European Patent Application EP 4 491 720 A1, published January 15, 2025. Title: COMPOSITIONS AND METHODS FOR INCREASING DELETION EFFICIENCY OF NUCLEIC ACID SEGMENT BY MODULATION OF NHEJ REPAIR PATHWAY. Applicant: GenKOre Co., Ltd. The sequence listing filed with the application follows.

SEQUENCE LISTING (473 sequences)

SEQ ID NO: 1 - protein, 557 aa, unidentified
  source 1..557: note = TnpB
MGEKSSRRRRNGKSGAWTAAITSCVGGKMAKNTITKTLKLRIVRPYNSAEVEKIVADEKNNREKIALEKNKDKVKEACSKHLKVAAYCTTQVERNACLFCKARKLDDKFYQKLRGQFPDAVFWQEISEIFRQLQKQAAEIYNQSLIELYYEIFIKGKGIANASSVEHYLSDVCYTRAAELFKNAAIASGLRSKIKSNFRLKELKNMKSGLPTTKSDNFPIPLVKQKGGQYTGFEISNHNSDFIIKIPFGRWQVKKEIDKYRPWEKFDFEQVQKSPKPISLLLSTQRRKRNKGWSKDEGTEAEIKKVMNGDYQTSYIEVKRGSKIGEKSAWMLNLSIDVPKIDKGVDPSIIGGIDVGVKSPLVCAINNAFSRYSISDNDLFHFNKKMFARRRILLKKNRHKRAGHGAKNKLKPITILTEKSERFRKKLIERWACEIADFFIKNKVGTVQMENLESMKRKEDSYFNIRLRGFWPYAEMQNKIEFKLKQYGIEIRKVAPNNTSKTCSKCGHLNNYFNFEYRKKNKFPHFKCEKCNFKENADYNAALNISNPKLKSTKEEP

SEQ ID NO: 2 - protein, 555 aa, synthetic construct
  source 1..555: note = TnpB-v1
MEKRINKIRKKLSADNATKPVSRSGPMAKNTITKTLKLRIVRPYNSAEVEKIVADEKNNREKIALEKNKDKVKEACSKHLKVAAYCTTQVERNACLFCKARKLDDKFYQKLRGQFPDAVFWQEISEIFRQLQKQAAEIYNQSLIELYYEIFIKGKGIANASSVEHYLSDVCYTRAAELFKNAAIASGLRSKIKSNFRLKELKNMKSGLPTTKSDNFPIPLVKQKGGQYTGFEISNHNSDFIIKIPFGRWQVKKEIDKYRPWEKFDFEQVQKSPKPISLLLSTQRRKRNKGWSKDEGTEAEIKKVMNGDYQTSYIEVKRGSKIGEKSAWMLNLSIDVPKIDKGVDPSIIGGIDVGVKSPLVCAINNAFSRYSISDNDLFHFNKKMFARRRILLKKNRHKRAGHGAKNKLKPITILTEKSERFRKKLIERWACEIADFFIKNKVGTVQMENLESMKRKEDSYFNIRLRGFWPYAEMQNKIEFKLKQYGIEIRKVAPNNTSKTCSKCGHLNNYFNFEYRKKNKFPHFKCEKCNFKENADYNAALNISNPKLKSTKEEP

SEQ ID NO: 3 - protein, 557 aa, synthetic construct
  source 1..557: note = TnpB-v2
MAGGPGAGSAAPVSSTSSLPLAALNMRVMAKNTITKTLKLRIVRPYNSAEVEKIVADEKNNREKIALEKNKDKVKEACSKHLKVAAYCTTQVERNACLFCKARKLDDKFYQKLRGQFPDAVFWQEISEIFRQLQKQAAEIYNQSLIELYYEIFIKGKGIANASSVEHYLSDVCYTRAAELFKNAAIASGLRSKIKSNFRLKELKNMKSGLPTTKSDNFPIPLVKQKGGQYTGFEISNHNSDFIIKIPFGRWQVKKEIDKYRPWEKFDFEQVQKSPKPISLLLSTQRRKRNKGWSKDEGTEAEIKKVMNGDYQTSYIEVKRGSKIGEKSAWMLNLSIDVPKIDKGVDPSIIGGIDVGVKSPLVCAINNAFSRYSISDNDLFHFNKKMFARRRILLKKNRHKRAGHGAKNKLKPITILTEKSERFRKKLIERWACEIADFFIKNKVGTVQMENLESMKRKEDSYFNIRLRGFWPYAEMQNKIEFKLKQYGIEIRKVAPNNTSKTCSKCGHLNNYFNFEYRKKNKFPHFKCEKCNFKENADYNAALNISNPKLKSTKEEP

SEQ ID NO: 4 - protein, 555 aa, synthetic construct
  source 1..555: note = TnpB-v3
MAGGPGAGSAAPVSSTSSLPLAALNMMAKNTITKTLKLRIVRPYNSAEVEKIVADEKNNREKIALEKNKDKVKEACSKHLKVAAYCTTQVERNACLFCKARKLDDKFYQKLRGQFPDAVFWQEISEIFRQLQKQAAEIYNQSLIELYYEIFIKGKGIANASSVEHYLSDVCYTRAAELFKNAAIASGLRSKIKSNFRLKELKNMKSGLPTTKSDNFPIPLVKQKGGQYTGFEISNHNSDFIIKIPFGRWQVKKEIDKYRPWEKFDFEQVQKSPKPISLLLSTQRRKRNKGWSKDEGTEAEIKKVMNGDYQTSYIEVKRGSKIGEKSAWMLNLSIDVPKIDKGVDPSIIGGIDVGVKSPLVCAINNAFSRYSISDNDLFHFNKKMFARRRILLKKNRHKRAGHGAKNKLKPITILTEKSERFRKKLIERWACEIADFFIKNKVGTVQMENLESMKRKEDSYFNIRLRGFWPYAEMQNKIEFKLKQYGIEIRKVAPNNTSKTCSKCGHLNNYFNFEYRKKNKFPHFKCEKCNFKENADYNAALNISNPKLKSTKEEP

SEQ ID NO: 5 - protein, 529 aa, synthetic construct
  source 1..529: note = Wild-type Cas12f1
MAKNTITKTLKLRIVRPYNSAEVEKIVADEKNNREKIALEKNKDKVKEACSKHLKVAAYCTTQVERNACLFCKARKLDDKFYQKLRGQFPDAVFWQEISEIFRQLQKQAAEIYNQSLIELYYEIFIKGKGIANASSVEHYLSDVCYTRAAELFKNAAIASGLRSKIKSNFRLKELKNMKSGLPTTKSDNFPIPLVKQKGGQYTGFEISNHNSDFIIKIPFGRWQVKKEIDKYRPWEKFDFEQVQKSPKPISLLLSTQRRKRNKGWSKDEGTEAEIKKVMNGDYQTSYIEVKRGSKIGEKSAWMLNLSIDVPKIDKGVDPSIIGGIDVGVKSPLVCAINNAFSRYSISDNDLFHFNKKMFARRRILLKKNRHKRAGHGAKNKLKPITILTEKSERFRKKLIERWACEIADFFIKNKVGTVQMENLESMKRKEDSYFNIRLRGFWPYAEMQNKIEFKLKQYGIEIRKVAPNNTSKTCSKCGHLNNYFNFEYRKKNKFPHFKCEKCNFKENADYNAALNISNPKLKSTKEEP

SEQ ID NO: 6 - DNA, 1671 bp, synthetic construct
  source 1..1671: mol_type = other DNA; note = Human codon-optimized TnpB
atgggggagaaaagttcccgccgccgacggaatggaaaaagcggtgcgtggactgctgctataacaagctgtgttgggggtaagatggccaagaacacaattacaaagacactgaagctgaggatcgtgagaccatacaacagcgctgaggtcgagaagattgtggctgatgaaaagaacaacagggaaaagatcgccctcgagaagaacaaggataaggtgaaggaggcctgctctaagcacctgaaagtggccgcctactgcaccacacaggtggagaggaacgcctgtctgttttgtaaagctcggaagctggatgataagttttaccagaagctgcggggccagttccccgatgccgtcttttggcaggagattagcgagatcttcagacagctgcagaagcaggccgccgagatctacaaccagagcctgatcgagctctactacgagatcttcatcaagggcaagggcattgccaacgcctcctccgtggagcactacctgagcgacgtgtgctacacaagagccgccgagctctttaagaacgccgctatcgcttccgggctgaggagcaagattaagagtaacttccggctcaaggagctgaagaacatgaagagcggcctgcccactacaaagagcgacaacttcccaattccactggtgaagcagaaggggggccagtacacagggttcgagatttccaaccacaacagcgactttattattaagatcccctttggcaggtggcaggtcaagaaggagattgacaagtacaggccctgggagaagtttgatttcgagcaggtgcagaagagccccaagcctatttccctgctgctgtccacacagcggcggaagaggaacaaggggtggtctaaggatgaggggaccgaggccgagattaagaaagtgatgaacggcgactaccagacaagctacatcgaggtcaagcggggcagtaagattggcgagaagagcgcctggatgctgaacctgagcattgacgtgccaaagattgataagggcgtggatcccagcatcatcggagggatcgatgtgggggtcaagagccccctcgtgtgcgccatcaacaacgccttcagcaggtacagcatctccgataacgacctgttccactttaacaagaagatgttcgcccggcggaggattttgctcaagaagaaccggcacaagcgggccggacacggggccaagaacaagctcaagcccatcactatcctgaccgagaagagcgagaggttcaggaagaagctcatcgagagatgggcctgcgagatcgccgatttctttattaagaacaaggtcggaacagtgcagatggagaacctcgagagcatgaagaggaaggaggattcctacttcaacattcggctgagggggttctggccctacgctgagatgcagaacaagattgagtttaagctgaagcagtacgggattgagatccggaaggtggcccccaacaacaccagcaagacctgcagcaagtgcgggcacctcaacaactacttcaacttcgagtaccggaagaagaacaagttcccacacttcaagtgcgagaagtgcaactttaaggagaacgccgattacaacgccgccctgaacatcagcaaccctaagctgaagagcactaaggaggagccc

SEQ ID NO: 7 - DNA, 1666 bp, synthetic construct
  source 1..1666: mol_type = other DNA; note = Human codon-optimized TnpB-V1
atggaaaagagaatcaacaagatcaggaagaagctgagcgccgacaacgccaccaagcctgtgtctaggagtggcccccatggccaagaacacaattacaaagacactgaagctgaggatcgtgagaccatacaacagcgctgaggtcgagaagattgtggctgatgaaaagaacaacagggaaaagatcgccctcgagaagaacaaggataaggtgaaggaggcctgctctaagcacctgaaagtggccgcctactgcaccacacaggtggagaggaacgcctgtctgttttgtaaagctcggaagctggatgataagttttaccagaagctgcggggccagttccccgatgccgtcttttggcaggagattagcgagatcttcagacagctgcagaagcaggccgccgagatctacaaccagagcctgatcgagctctactacgagatcttcatcaagggcaagggcattgccaacgcctcctccgtggagcactacctgagcgacgtgtgctacacaagagccgccgagctctttaagaacgccgctatcgcttccgggctgaggagcaagattaagagtaacttccggctcaaggagctgaagaacatgaagagcggcctgcccactacaaagagcgacaacttcccaattccactggtgaagcagaaggggggccagtacacagggttcgagatttccaaccacaacagcgactttattattaagatcccctttggcaggtggcaggtcaagaaggagattgacaagtacaggccctgggagaagtttgatttcgagcaggtgcagaagagccccaagcctatttccctgctgctgtccacacagcggcggaagaggaacaaggggtggtctaaggatgaggggaccgaggccgagattaagaaagtgatgaacggcgactaccagacaagctacatcgaggtcaagcggggcagtaagattggcgagaagagcgcctggatgctgaacctgagcattgacgtgccaaagattgataagggcgtggatcccagcatcatcggagggatcgatgtgggggtcaagagccccctcgtgtgcgccatcaacaacgccttcagcaggtacagcatctccgataacgacctgttccactttaacaagaagatgttcgcccggcggaggattttgctcaagaagaaccggcacaagcgggccggacacggggccaagaacaagctcaagcccatcactatcctgaccgagaagagcgagaggttcaggaagaagctcatcgagagatgggcctgcgagatcgccgatttctttattaagaacaaggtcggaacagtgcagatggagaacctcgagagcatgaagaggaaggaggattcctacttcaacattcggctgagggggttctggccctacgctgagatgcagaacaagattgagtttaagctgaagcagtacgggattgagatccggaaggtggcccccaacaacaccagcaagacctgcagcaagtgcgggcacctcaacaactacttcaacttcgagtaccggaagaagaacaagttcccacacttcaagtgcgagaagtgcaactttaaggagaacgccgattacaacgccgccctgaacatcagcaaccctaagctgaagagcactaaggaggagccc

SEQ ID NO: 8 - DNA, 1671 bp, synthetic construct
  source 1..1671: mol_type = other DNA; note = Human codon-optimized TnpB-V2
atggctggcggaccaggcgcaggtagtgctgcgccagtttcttcaacttcctccctgcccctggctgcgcttaacatgcgcgtgatggccaagaacacaattacaaagacactgaagctgaggatcgtgagaccatacaacagcgctgaggtcgagaagattgtggctgatgaaaagaacaacagggaaaagatcgccctcgagaagaacaaggataaggtgaaggaggcctgctctaagcacctgaaagtggccgcctactgcaccacacaggtggagaggaacgcctgtctgttttgtaaagctcggaagctggatgataagttttaccagaagctgcggggccagttccccgatgccgtcttttggcaggagattagcgagatcttcagacagctgcagaagcaggccgccgagatctacaaccagagcctgatcgagctctactacgagatcttcatcaagggcaagggcattgccaacgcctcctccgtggagcactacctgagcgacgtgtgctacacaagagccgccgagctctttaagaacgccgctatcgcttccgggctgaggagcaagattaagagtaacttccggctcaaggagctgaagaacatgaagagcggcctgcccactacaaagagcgacaacttcccaattccactggtgaagcagaaggggggccagtacacagggttcgagatttccaaccacaacagcgactttattattaagatcccctttggcaggtggcaggtcaagaaggagattgacaagtacaggccctgggagaagtttgatttcgagcaggtgcagaagagccccaagcctatttccctgctgctgtccacacagcggcggaagaggaacaaggggtggtctaaggatgaggggaccgaggccgagattaagaaagtgatgaacggcgactaccagacaagctacatcgaggtcaagcggggcagtaagattggcgagaagagcgcctggatgctgaacctgagcattgacgtgccaaagattgataagggcgtggatcccagcatcatcggagggatcgatgtgggggtcaagagccccctcgtgtgcgccatcaacaacgccttcagcaggtacagcatctccgataacgacctgttccactttaacaagaagatgttcgcccggcggaggattttgctcaagaagaaccggcacaagcgggccggacacggggccaagaacaagctcaagcccatcactatcctgaccgagaagagcgagaggttcaggaagaagctcatcgagagatgggcctgcgagatcgccgatttctttattaagaacaaggtcggaacagtgcagatggagaacctcgagagcatgaagaggaaggaggattcctacttcaacattcggctgagggggttctggccctacgctgagatgcagaacaagattgagtttaagctgaagcagtacgggattgagatccggaaggtggcccccaacaacaccagcaagacctgcagcaagtgcgggcacctcaacaactacttcaacttcgagtaccggaagaagaacaagttcccacacttcaagtgcgagaagtgcaactttaaggagaacgccgattacaacgccgccctgaacatcagcaaccctaagctgaagagcactaaggaggagccc

SEQ ID NO: 9 - DNA, 1665 bp, synthetic construct
  source 1..1665: mol_type = other DNA; note = Human codon-optimized TnpB-V3
atggctggcggaccaggcgcaggtagtgctgcgccagtttcttcaacttcctccctgcccctggctgcgcttaacatgatggccaagaacacaattacaaagacactgaagctgaggatcgtgagaccatacaacagcgctgaggtcgagaagattgtggctgatgaaaagaacaacagggaaaagatcgccctcgagaagaacaaggataaggtgaaggaggcctgctctaagcacctgaaagtggccgcctactgcaccacacaggtggagaggaacgcctgtctgttttgtaaagctcggaagctggatgataagttttaccagaagctgcggggccagttccccgatgccgtcttttggcaggagattagcgagatcttcagacagctgcagaagcaggccgccgagatctacaaccagagcctgatcgagctctactacgagatcttcatcaagggcaagggcattgccaacgcctcctccgtggagcactacctgagcgacgtgtgctacacaagagccgccgagctctttaagaacgccgctatcgcttccgggctgaggagcaagattaagagtaacttccggctcaaggagctgaagaacatgaagagcggcctgcccactacaaagagcgacaacttcccaattccactggtgaagcagaaggggggccagtacacagggttcgagatttccaaccacaacagcgactttattattaagatcccctttggcaggtggcaggtcaagaaggagattgacaagtacaggccctgggagaagtttgatttcgagcaggtgcagaagagccccaagcctatttccctgctgctgtccacacagcggcggaagaggaacaaggggtggtctaaggatgaggggaccgaggccgagattaagaaagtgatgaacggcgactaccagacaagctacatcgaggtcaagcggggcagtaagattggcgagaagagcgcctggatgctgaacctgagcattgacgtgccaaagattgataagggcgtggatcccagcatcatcggagggatcgatgtgggggtcaagagccccctcgtgtgcgccatcaacaacgccttcagcaggtacagcatctccgataacgacctgttccactttaacaagaagatgttcgcccggcggaggattttgctcaagaagaaccggcacaagcgggccggacacggggccaagaacaagctcaagcccatcactatcctgaccgagaagagcgagaggttcaggaagaagctcatcgagagatgggcctgcgagatcgccgatttctttattaagaacaaggtcggaacagtgcagatggagaacctcgagagcatgaagaggaaggaggattcctacttcaacattcggctgagggggttctggccctacgctgagatgcagaacaagattgagtttaagctgaagcagtacgggattgagatccggaaggtggcccccaacaacaccagcaagacctgcagcaagtgcgggcacctcaacaactacttcaacttcgagtaccggaagaagaacaagttcccacacttcaagtgcgagaagtgcaactttaaggagaacgccgattacaacgccgccctgaacatcagcaaccctaagctgaagagcactaaggaggagccc

SEQ ID NO: 10 - DNA, 1587 bp, synthetic construct
  source 1..1587: mol_type = other DNA; note = Human codon-optimized Cas12f1
atggccaagaacacaattacaaagacactgaagctgaggatcgtgagaccatacaacagcgctgaggtcgagaagattgtggctgatgaaaagaacaacagggaaaagatcgccctcgagaagaacaaggataaggtgaaggaggcctgctctaagcacctgaaagtggccgcctactgcaccacacaggtggagaggaacgcctgtctgttttgtaaagctcggaagctggatgataagttttaccagaagctgcggggccagttccccgatgccgtcttttggcaggagattagcgagatcttcagacagctgcagaagcaggccgccgagatctacaaccagagcctgatcgagctctactacgagatcttcatcaagggcaagggcattgccaacgcctcctccgtggagcactacctgagcgacgtgtgctacacaagagccgccgagctctttaagaacgccgctatcgcttccgggctgaggagcaagattaagagtaacttccggctcaaggagctgaagaacatgaagagcggcctgcccactacaaagagcgacaacttcccaattccactggtgaagcagaaggggggccagtacacagggttcgagatttccaaccacaacagcgactttattattaagatcccctttggcaggtggcaggtcaagaaggagattgacaagtacaggccctgggagaagtttgatttcgagcaggtgcagaagagccccaagcctatttccctgctgctgtccacacagcggcggaagaggaacaaggggtggtctaaggatgaggggaccgaggccgagattaagaaagtgatgaacggcgactaccagacaagctacatcgaggtcaagcggggcagtaagattggcgagaagagcgcctggatgctgaacctgagcattgacgtgccaaagattgataagggcgtggatcccagcatcatcggagggatcgatgtgggggtcaagagccccctcgtgtgcgccatcaacaacgccttcagcaggtacagcatctccgataacgacctgttccactttaacaagaagatgttcgcccggcggaggattttgctcaagaagaaccggcacaagcgggccggacacggggccaagaacaagctcaagcccatcactatcctgaccgagaagagcgagaggttcaggaagaagctcatcgagagatgggcctgcgagatcgccgatttctttattaagaacaaggtcggaacagtgcagatggagaacctcgagagcatgaagaggaaggaggattcctacttcaacattcggctgagggggttctggccctacgctgagatgcagaacaagattgagtttaagctgaagcagtacgggattgagatccggaaggtggcccccaacaacaccagcaagacctgcagcaagtgcgggcacctcaacaactacttcaacttcgagtaccggaagaagaacaagttcccacacttcaagtgcgagaagtgcaactttaaggagaacgccgattacaacgccgccctgaacatcagcaaccctaagctgaagagcactaaggaggagccc

SEQ ID NO: 11 - RNA, 161 nt, synthetic construct
  source 1..161: mol_type = other RNA; note = Wild-type tracrRNA for TnpB or Cas12f1 gRNA
cttcactgataaagtggagaaccgcttcaccaaaagctgtcccttaggggattagaacttgagtgaaggtgggctgcttgcatcagcctaatgtcgagaagtgctttcttcggaaagtaaccctcgaaacaaattcatttttcctctccaattctgcacaa

SEQ ID NO: 12 - RNA, 37 nt, synthetic construct
  source 1..37: mol_type = other RNA; note = Wild-type crRNA for TnpB or Cas12f1 gRNA
gttgcagaacccgaatagacgaatgaaggaatgcaac

SEQ ID NO: 13 - RNA, 222 nt, synthetic construct
  source 1..222: mol_type = other RNA; note = Canonical sgRNA for TnpB or Cas12f1
  misc_feature 203..222: note = n is a, c, g or u
cttcactgataaagtggagaaccgcttcaccaaaagctgtcccttaggggattagaacttgagtgaaggtgggctgcttgcatcagcctaatgtcgagaagtgctttcttcggaaagtaaccctcgaaacaaattcatttttcctctccaattctgcacaagaaagttgcagaacccgaatagacgaatgaaggaatgcaacnnnnnnnnnnnnnnnnnnnn

SEQ ID NO: 14 - RNA, 20 nt, synthetic construct
  source 1..20: mol_type = other RNA; note = Xa of Formula (I)
cttcactgataaagtggaga

SEQ ID NO: 15 - RNA, 19 nt, synthetic construct
  source 1..19: mol_type = other RNA; note = Xa of Formula (I)
ttcactgataaagtggaga

SEQ ID NO: 16 - RNA, 18 nt, synthetic construct
  source 1..18: mol_type = other RNA; note = Xa of Formula (I)
tcactgataaagtggaga

SEQ ID NO: 17 - RNA, 17 nt, synthetic construct
  source 1..17: mol_type = other RNA; note = Xa of Formula (I)
cactgataaagtggaga

SEQ ID NO: 18 - RNA, 16 nt, synthetic construct
  source 1..16: mol_type = other RNA; note = Xa of Formula (I)
actgataaagtggaga

SEQ ID NO: 19 - RNA, 15 nt, synthetic construct
  source 1..15: mol_type = other RNA; note = Xa of Formula (I)
ctgataaagtggaga

SEQ ID NO: 20 - RNA, 14 nt, synthetic construct
  source 1..14: mol_type = other RNA; note = Xa of Formula (I)
tgataaagtggaga

SEQ ID NO: 21 - RNA, 13 nt, synthetic construct
  source 1..13: mol_type = other RNA; note = Xa of Formula (I)
gataaagtggaga

SEQ ID NO: 22 - RNA, 12 nt, synthetic construct
  source 1..12: mol_type = other RNA; note = Xa of Formula (I)
ataaagtggaga

SEQ ID NO: 23 - RNA, 11 nt, synthetic construct
  source 1..11: mol_type = other RNA; note = Xa of Formula (I)
taaagtggaga

SEQ ID NO: 24 - RNA, 10 nt, synthetic construct
  source 1..10: mol_type = other RNA; note = Xa of Formula (I)
aaagtggaga

SEQ ID NO: 25 - RNA, 13 nt, synthetic construct
  source 1..13: mol_type = other RNA; note = Xb1 of Formula (I)
caaaagctgtccc

SEQ ID NO: 26 - RNA, 12 nt, synthetic construct
  source 1..12: mol_type = other RNA; note = Xb1 of Formula (I)
caaaagctgtcc

SEQ ID NO: 27 - RNA, 11 nt, synthetic construct
  source 1..11: mol_type = other RNA; note = Xb1 of Formula (I)
caaaagctgtc

SEQ ID NO: 28 - RNA, 10 nt, synthetic construct
  source 1..10: mol_type = other RNA; note = Xb1 of Formula (I)
caaaagctgt

SEQ ID NO: 29 - RNA, 14 nt, synthetic construct
  source 1..14: mol_type = other RNA; note = Xb2 of Formula (I)
gggattagaacttg

SEQ ID NO: 30 - RNA, 13 nt, synthetic construct
  source 1..13: mol_type = other RNA; note = Xb2 of Formula (I)
ggattagaacttg

SEQ ID NO: 31 - RNA, 12 nt, synthetic construct
  source 1..12: mol_type = other RNA; note = Xb2 of Formula (I)
gattagaacttg

SEQ ID NO: 32 - RNA, 11 nt, synthetic construct
  source 1..11: mol_type = other RNA; note = Xb2 of Formula (I)
attagaacttg

SEQ ID NO: 33 - RNA, 10 nt, synthetic construct
  source 1..10: mol_type = other RNA; note = Xb2 of Formula (I)
ttagaacttg

SEQ ID NO: 34 - RNA, 31 nt, synthetic construct
  source 1..31: mol_type = other RNA; note = Xb1-UUAG-Xb2 of Formula (I)
caaaagctgtcccttaggggattagaacttg

SEQ ID NO: 35 - RNA, 25 nt, synthetic construct
  source 1..25: mol_type = other RNA; note = Xb1-UUAG-Xb2 of Formula (I)
caaaagctgtttagattagaacttg

SEQ ID NO: 36 - RNA, 20 nt, synthetic construct
  source 1..20: mol_type = other RNA; note = Xb1-UUAG-Xb2 of Formula (I)
caaaagctttagagaacttg

SEQ ID NO: 37 - RNA, 18 nt, synthetic construct
  source 1..18: mol_type = other RNA; note = Xb1-UUAG-Xb2 of Formula (I)
caaaagcttaggaacttg

SEQ ID NO: 38 - RNA, 10 nt, synthetic construct
  source 1..10: mol_type = other RNA; note = Xb1-UUAG-Xb2 of Formula (I)
caattagttg

SEQ ID NO: 39 - RNA, 28 nt, synthetic construct
  source 1..28: mol_type = other RNA; note = Xc1 of Formula (I)
ttcatttttcctctccaattctgcacaa

SEQ ID NO: 40 - RNA, 27 nt, synthetic construct
  source 1..27: mol_type = other RNA; note = Xc1 of Formula (I)
ttcatttttcctctccaattctgcaca

SEQ ID NO: 41 - RNA, 26 nt, synthetic construct
  source 1..26: mol_type = other RNA; note = Xc1 of Formula (I)
ttcatttttcctctccaattctgcac

SEQ ID NO: 42 - RNA, 25 nt, synthetic construct
  source 1..25: mol_type = other RNA; note = Xc1 of Formula (I)
ttcatttttcctctccaattctgca

SEQ ID NO: 43 - RNA, 24 nt, synthetic construct
  source 1..24: mol_type = other RNA; note = Xc1 of Formula (I)
ttcatttttcctctccaattctgc

SEQ ID NO: 44 - RNA, 23 nt, synthetic construct
  source 1..23: mol_type = other RNA; note = Xc1 of Formula (I)
ttcatttttcctctccaattctg

SEQ ID NO: 45 - RNA, 22 nt, synthetic construct
  source 1..22: mol_type = other RNA; note = Xc1 of Formula (I)
ttcatttttcctctccaattct

SEQ ID NO: 46 - RNA, 21 nt, synthetic construct
  source 1..21: mol_type = other RNA; note = Xc1 of Formula (I)
ttcatttttcctctccaattc

SEQ ID NO: 47 - RNA, 20 nt, synthetic construct
  source 1..20: mol_type = other RNA; note = Xc1 of Formula (I)
ttcatttttcctctccaatt

SEQ ID NO: 48 - RNA, 19 nt, synthetic construct
  source 1..19: mol_type = other RNA; note = Xc1 of Formula (I)
ttcatttttcctctccaat

SEQ ID NO: 49 - RNA, 18 nt, synthetic construct
  source 1..18: mol_type = other RNA; note = Xc1 of Formula (I)
ttcatttttcctctccaa

SEQ ID NO: 50 - RNA, 17 nt, synthetic construct
  source 1..17: mol_type = other RNA; note = Xc1 of Formula (I)
ttcatttttcctctcca

SEQ ID NO: 51 - RNA, 16 nt, synthetic construct
  source 1..16: mol_type = other RNA; note = Xc1 of Formula (I)
ttcatttttcctctcc

SEQ ID NO: 52 - RNA, 15 nt, synthetic construct
  source 1..15: mol_type = other RNA; note = Xc1 of Formula (I)
ttcatttttcctctc

SEQ ID NO: 53 - RNA, 14 nt, synthetic construct
  source 1..14: mol_type = other RNA; note = Xc1 of Formula (I)
ttcatttttcctct

SEQ ID NO: 54 - RNA, 13 nt, synthetic construct
  source 1..13: mol_type = other RNA; note = Xc1 of Formula (I)
ttcatttttcctc

SEQ ID NO: 55 - RNA, 12 nt, synthetic construct
  source 1..12: mol_type = other RNA; note = Xc1 of Formula (I)
ttcatttttcct

SEQ ID NO: 56 - RNA, 11 nt, synthetic construct
  source 1..11: mol_type = other RNA; note = Xc1 of Formula (I)
ttcatttttcc

SEQ ID NO: 57 - RNA, 10 nt, synthetic construct
  source 1..10: mol_type = other RNA; note = Xc1 of Formula (I)
ttcatttttc

SEQ ID NO: 58 - RNA, 27 nt, synthetic construct
  source 1..27: mol_type = other RNA; note = Xc2 of Formula (I)
gttgcagaacccgaatagacgaatgaa

SEQ ID NO: 59 - RNA, 26 nt, synthetic construct
  source 1..26: mol_type = other RNA; note = Xc2 of Formula (I)
ttgcagaacccgaatagacgaatgaa

SEQ ID NO: 60 - RNA, 25 nt, synthetic construct
  source 1..25: mol_type = other RNA; note = Xc2 of Formula (I)
tgcagaacccgaatagacgaatgaa

SEQ ID NO: 61 - RNA, 24 nt, synthetic construct
  source 1..24: mol_type = other RNA; note = Xc2 of Formula (I)
gcagaacccgaatagacgaatgaa

SEQ ID NO: 62 - RNA, 23 nt, synthetic construct
  source 1..23: mol_type = other RNA; note = Xc2 of Formula (I)
cagaacccgaatagacgaatgaa

SEQ ID NO: 63 - RNA, 22 nt, synthetic construct
  source 1..22: mol_type = other RNA; note = Xc2 of Formula (I)
agaacccgaatagacgaatgaa

SEQ ID NO: 64 - RNA, 21 nt, synthetic construct
  source 1..21: mol_type = other RNA; note = Xc2 of Formula (I)
gaacccgaatagacgaatgaa

SEQ ID NO: 65 - RNA, 20 nt, synthetic construct
  source 1..20: mol_type = other RNA; note = Xc2 of Formula (I)
aacccgaatagacgaatgaa

SEQ ID NO: 66 - RNA, 19 nt, synthetic construct
  source 1..19: mol_type = other RNA; note = Xc2 of Formula (I)
acccgaatagacgaatgaa

SEQ ID NO: 67 - RNA, 18 nt, synthetic construct
  source 1..18: mol_type = other RNA; note = Xc2 of Formula (I)
cccgaatagacgaatgaa

SEQ ID NO: 68 - RNA, 17 nt, synthetic construct
  source 1..17: mol_type = other RNA; note = Xc2 of Formula (I)
ccgaatagacgaatgaa

SEQ ID NO: 69 - RNA, 16 nt, synthetic construct
  source 1..16: mol_type = other RNA; note = Xc2 of Formula (I)
cgaatagacgaatgaa

SEQ ID NO: 70 - RNA, 15 nt, synthetic construct
  source 1..15: mol_type = other RNA; note = Xc2 of Formula (I)
gaatagacgaatgaa

SEQ ID NO: 71 - RNA, 14 nt, synthetic construct
  source 1..14: mol_type = other RNA; note = Xc2 of Formula (I)
aatagacgaatgaa

SEQ ID NO: 72 - RNA, 13 nt, synthetic construct
  source 1..13: mol_type = other RNA; note = Xc2 of Formula (I)
atagacgaatgaa

SEQ ID NO: 73 - RNA, 12 nt, synthetic construct
  source 1..12: mol_type = other RNA; note = Xc2 of Formula (I)
tagacgaatgaa

SEQ ID NO: 74 - RNA, 11 nt, synthetic construct
  source 1..11: mol_type = other RNA; note = Xc2 of Formula (I)
agacgaatgaa

SEQ ID NO: 75 - RNA, 10 nt, synthetic construct
  source 1..10: mol_type = other RNA; note = Xc2 of Formula (I)
gacgaatgaa

SEQ ID NO: 76 - RNA, 10 nt, synthetic construct
  source 1..10: mol_type = other RNA; note = Linker (Lk)
ttcgaaagaa

SEQ ID NO: 77 - RNA, 12 nt, synthetic construct
  source 1..12: mol_type = other RNA; note = Linker (Lk)
ttcagaaatgaa

SEQ ID NO: 78 - RNA, 14 nt, synthetic construct
  source 1..14: mol_type = other RNA; note = Linker (Lk)
ttcatgaaaatgaa

SEQ ID NO: 79 - RNA, 16 nt, synthetic construct
  source 1..16: mol_type = other RNA; note = Linker (Lk)
ttcattgaaaaatgaa

SEQ ID NO: 80 - RNA, 59 nt, synthetic construct
  source 1..59: mol_type = other RNA; note = Xc1-Lk-Xc2 of Formula (I)
ttcagtgctcctctccaattctgcacaagaaagttgcagaacccgaatagagcaatgaa

SEQ ID NO: 81 - RNA, 46 nt, synthetic construct
  source 1..46: mol_type = other RNA; note = Xc1-Lk-Xc2 of Formula (I)
ttcagtgctcctctccaattcgaaagaacccgaatagagcaatgaa

SEQ ID NO: 82 - RNA, 34 nt, synthetic construct
  source 1..34: mol_type = other RNA; note = Xc1-Lk-Xc2 of Formula (I)
ttcagtgctcctctcgaaagaatagagcaatgaa

SEQ ID NO: 83 - RNA, 22 nt, synthetic construct
  source 1..22: mol_type = other RNA; note = Xc1-Lk-Xc2 of Formula (I)
ttcagtgctgaaaagcaatgaa

SEQ ID NO: 84 - RNA, 18 nt, synthetic construct
  source 1..18: mol_type = other RNA; note = Xc1-Lk-Xc2 of Formula (I)
ttcatttgaaagaatgaa

SEQ ID NO: 85 - RNA, 14 nt, synthetic construct
  source 1..14: mol_type = other RNA; note = Xc1-Lk-Xc2 of Formula (I)
ttcatgaaaatgaa

SEQ ID NO: 86 - RNA, 10 nt, synthetic construct
  source 1..10: mol_type = other RNA; note = Xc1-Lk-Xc2 of Formula (I)
ttcgaaagaa

SEQ ID NO: 87 - RNA, 161 nt, synthetic construct
  source 1..161: mol_type = other RNA; note = Engineered tracrRNA for TnpB or Cas12f1 gRNA (MS1)
cttcactgataaagtggagaaccgcttcaccaaaagctgtcccttaggggattagaacttgagtgaaggtgggctgcttgcatcagcctaatgtcgagaagtgctttcttcggaaagtaaccctcgaaacaaattcagtgctcctctccaattctgcacaa

SEQ ID NO: 88 - RNA, 154 nt, synthetic construct
  source 1..154: mol_type = other RNA; note = Engineered tracrRNA for TnpB or Cas12f1 gRNA (MS1/MS3-1)
gataaagtggagaaccgcttcaccaaaagctgtcccttaggggattagaacttgagtgaaggtgggctgcttgcatcagcctaatgtcgagaagtgctttcttcggaaagtaaccctcgaaacaaattcagtgctcctctccaattctgcacaa

SEQ ID NO: 89 - RNA, 147 nt, synthetic construct
  source 1..147: mol_type = other RNA; note = Engineered tracrRNA for TnpB or Cas12f1 gRNA (MS1/MS3-2)
tggagaaccgcttcaccaaaagctgtcccttaggggattagaacttgagtgaaggtgggctgcttgcatcagcctaatgtcgagaagtgctttcttcggaaagtaaccctcgaaacaaattcagtgctcctctccaattctgcacaa

SEQ ID NO: 90 - RNA, 141 nt, synthetic construct
  source 1..141: mol_type = other RNA; note = Engineered tracrRNA for TnpB or Cas12f1 gRNA (MS1/MS3-3)
accgcttcaccaaaagctgtcccttaggggattagaacttgagtgaaggtgggctgcttgcatcagcctaatgtcgagaagtgctttcttcggaaagtaaccctcgaaacaaattcagtgctcctctccaattctgcacaa

SEQ ID NO: 91 - RNA, 154 nt, synthetic construct
  source 1..154: mol_type = other RNA; note = Engineered tracrRNA for TnpB or Cas12f1 gRNA (MS1/MS4*-1)
cttcactgataaagtggagaaccgcttcaccaaaagctgtcccttaggggattagaacttgagtgaaggtgggctgcttgcatcagcctaatgtcgagaagtgctttcttcggaaagtaaccctcgaaacaaattcagtgctcctctccaattc

SEQ ID NO: 92 - RNA, 148 nt, synthetic construct
  source 1..148: mol_type = other RNA; note = Engineered tracrRNA for TnpB or Cas12f1 gRNA (MS1/MS4*-2)
cttcactgataaagtggagaaccgcttcaccaaaagctgtcccttaggggattagaacttgagtgaaggtgggctgcttgcatcagcctaatgtcgagaagtgctttcttcggaaagtaaccctcgaaacaaattcagtgctcctctc

SEQ ID NO: 93 - RNA, 142 nt, synthetic construct
  source 1..142: mol_type = other RNA; note = Engineered tracrRNA for TnpB or Cas12f1 gRNA (MS1/MS4*-3)
cttcactgataaagtggagaaccgcttcaccaaaagctgtcccttaggggattagaacttgagtgaaggtgggctgcttgcatcagcctaatgtcgagaagtgctttcttcggaaagtaaccctcgaaacaaattcagtgct

SEQ ID NO: 94 - RNA, 155 nt, synthetic construct
  source 1..155: mol_type = other RNA; note = Engineered tracrRNA for TnpB or Cas12f1 gRNA (MS1/MS5-1)
cttcactgataaagtggagaaccgcttcaccaaaagctgtttagattagaacttgagtgaaggtgggctgcttgcatcagcctaatgtcgagaagtgctttcttcggaaagtaaccctcgaaacaaattcagtgctcctctccaattctgcacaa

SEQ ID NO: 95 - RNA, 148 nt, synthetic construct
  source 1..148: mol_type = other RNA; note = Engineered tracrRNA for TnpB or Cas12f1 gRNA (MS1/MS5-2)
cttcactgataaagtggagaaccgcttcaccaaaagcttaggaacttgagtgaaggtgggctgcttgcatcagcctaatgtcgagaagtgctttcttcggaaagtaaccctcgaaacaaattcagtgctcctctccaattctgcacaa

SEQ ID NO: 96 - RNA, 140 nt, synthetic construct
  source 1..140: mol_type = other RNA; note = Engineered tracrRNA for TnpB or Cas12f1 gRNA (MS1/MS5-3)
cttcactgataaagtggagaaccgcttcaccaattagttgagtgaaggtgggctgcttgcatcagcctaatgtcgagaagtgctttcttcggaaagtaaccctcgaaacaaattcagtgctcctctccaattctgcacaa

SEQ ID NO: 97 - RNA, 134 nt, synthetic construct
  source 1..134: mol_type = other RNA; note = Engineered tracrRNA for TnpB or Cas12f1 gRNA (MS1/MS3-3/MS4*-1)
accgcttcaccaaaagctgtcccttaggggattagaacttgagtgaaggtgggctgcttgcatcagcctaatgtcgagaagtgctttcttcggaaagtaaccctcgaaacaaattcagtgctcctctccaattc

SEQ ID NO: 98 - RNA, 128 nt, synthetic construct
  source 1..128: mol_type = other RNA; note = Engineered tracrRNA for TnpB or Cas12f1 gRNA (MS1/MS3-3/MS4*-2)
accgcttcaccaaaagctgtcccttaggggattagaacttgagtgaaggtgggctgcttgcatcagcctaatgtcgagaagtgctttcttcggaaagtaaccctcgaaacaaattcagtgctcctctc

SEQ ID NO: 99 - RNA, 122 nt, synthetic construct
  source 1..122: mol_type = other RNA; note = Engineered tracrRNA for TnpB or Cas12f1 gRNA (MS1/MS3-3/MS4*-3)
accgcttcaccaaaagctgtcccttaggggattagaacttgagtgaaggtgggctgcttgcatcagcctaatgtcgagaagtgctttcttcggaaagtaaccctcgaaacaaattcagtgct

SEQ ID NO: 100 - RNA, 142 nt, synthetic construct
  source 1..142: mol_type = other RNA; note = Engineered tracrRNA for TnpB or Cas12f1 gRNA (MS1/MS4*-2/MS5-1)
cttcactgataaagtggagaaccgcttcaccaaaagctgtttagattagaacttgagtgaaggtgggctgcttgcatcagcctaatgtcgagaagtgctttcttcggaaagtaaccctcgaaacaaattcagtgctcctctc

SEQ ID NO: 101 - RNA, 135 nt, synthetic construct
  source 1..135: mol_type = other RNA; note = Engineered tracrRNA for TnpB or Cas12f1 gRNA (MS1/MS4*-2/MS5-2)
cttcactgataaagtggagaaccgcttcaccaaaagcttaggaacttgagtgaaggtgggctgcttgcatcagcctaatgtcgagaagtgctttcttcggaaagtaaccctcgaaacaaattcagtgctcctctc

SEQ ID NO: 102 - RNA, 127 nt, synthetic construct
  source 1..127: mol_type = other RNA; note = Engineered tracrRNA for TnpB or Cas12f1 gRNA (MS1/MS4*-2/MS5-3)
cttcactgataaagtggagaaccgcttcaccaattagttgagtgaaggtgggctgcttgcatcagcctaatgtcgagaagtgctttcttcggaaagtaaccctcgaaacaaattcagtgctcctctc

SEQ ID NO: 103 - RNA, 135 nt, synthetic construct
  source 1..135: mol_type = other RNA; note = Engineered tracrRNA for TnpB or Cas12f1 gRNA (MS1/MS3-3/MS5-1)
accgcttcaccaaaagctgtttagattagaacttgagtgaaggtgggctgcttgcatcagcctaatgtcgagaagtgctttcttcggaaagtaaccctcgaaacaaattcagtgctcctctccaattctgcacaa

SEQ ID NO: 104 - RNA, 128 nt, synthetic construct
  source 1..128: mol_type = other RNA; note = Engineered tracrRNA for TnpB or Cas12f1 gRNA (MS1/MS3-3/MS5-2)
accgcttcaccaaaagcttaggaacttgagtgaaggtgggctgcttgcatcagcctaatgtcgagaagtgctttcttcggaaagtaaccctcgaaacaaattcagtgctcctctccaattctgcacaa

SEQ ID NO: 105 - RNA, 120 nt, synthetic construct
  source 1..120: mol_type = other RNA; note = Engineered tracrRNA for TnpB or Cas12f1 gRNA (MS1/MS3-3/MS5-3)
accgcttcaccaattagttgagtgaaggtgggctgcttgcatcagcctaatgtcgagaagtgctttcttcggaaagtaaccctcgaaacaaattcagtgctcctctccaattctgcacaa

SEQ ID NO: 106 - RNA, 107 nt, synthetic construct
  source 1..107: mol_type = other RNA; note = Engineered tracrRNA for TnpB or Cas12f1 gRNA (MS1/MS3-3/MS4*-2/MS5-3)
accgcttcaccaattagttgagtgaaggtgggctgcttgcatcagcctaatgtcgagaagtgctttcttcggaaagtaaccctcgaaacaaattcagtgctcctctc

SEQ ID NO: 107 - RNA, 140 nt, synthetic construct
  source 1..140: mol_type = other RNA; note = Engineered tracrRNA for TnpB or Cas12f1 gRNA (MF)
cttcactgataaagtggagaaccgcttcaccaaaagctgtcccttaggggattagaacttgagtgaaggtgggctgcttgcatcagcctaatgtcgagaagtgctttcttcggaaagtaaccctcgaaacaaattcattt

SEQ ID NO: 108 - RNA, 133 nt, synthetic construct
  source 1..133: mol_type = other RNA; note = Engineered tracrRNA for TnpB or Cas12f1 gRNA (MF/MS3-1)
gataaagtggagaaccgcttcaccaaaagctgtcccttaggggattagaacttgagtgaaggtgggctgcttgcatcagcctaatgtcgagaagtgctttcttcggaaagtaaccctcgaaacaaattcattt

SEQ ID NO: 109 - RNA, 126 nt, synthetic construct
  source 1..126: mol_type = other RNA; note = Engineered tracrRNA for TnpB or Cas12f1 gRNA (MF/MS3-2)
tggagaaccgcttcaccaaaagctgtcccttaggggattagaacttgagtgaaggtgggctgcttgcatcagcctaatgtcgagaagtgctttcttcggaaagtaaccctcgaaacaaattcattt

SEQ ID NO: 110 - RNA, 120 nt, synthetic construct
  source 1..120: mol_type = other RNA; note = Engineered tracrRNA for TnpB or Cas12f1 gRNA (MF/MS3-3)
accgcttcaccaaaagctgtcccttaggggattagaacttgagtgaaggtgggctgcttgcatcagcctaatgtcgagaagtgctttcttcggaaagtaaccctcgaaacaaattcattt

SEQ ID NO: 111 - RNA, 138 nt, synthetic construct
  source 1..138: mol_type = other RNA; note = Engineered tracrRNA for TnpB or Cas12f1 gRNA (MF/MS4-1)
cttcactgataaagtggagaaccgcttcaccaaaagctgtcccttaggggattagaacttgagtgaaggtgggctgcttgcatcagcctaatgtcgagaagtgctttcttcggaaagtaaccctcgaaacaaattcat

SEQ ID NO: 112 - RNA, 136 nt, synthetic construct
  source 1..136: mol_type = other RNA; note = Engineered tracrRNA for TnpB or Cas12f1 gRNA (MF/MS4-2)
cttcactgataaagtggagaaccgcttcaccaaaagctgtcccttaggggattagaacttgagtgaaggtgggctgcttgcatcagcctaatgtcgagaagtgctttcttcggaaagtaaccctcgaaacaaattc

SEQ ID NO: 113 - RNA, 133 nt, synthetic construct
  source 1..133: mol_type = other RNA; note = Engineered tracrRNA for TnpB or Cas12f1 gRNA (MF/MS4-3)
cttcactgataaagtggagaaccgcttcaccaaaagctgtcccttaggggattagaacttgagtgaaggtgggctgcttgcatcagcctaatgtcgagaagtgctttcttcggaaagtaaccctcgaaacaaa

SEQ ID NO: 114 - RNA, 134 nt, synthetic construct
  source 1..134: mol_type = other RNA; note = Engineered tracrRNA for TnpB or Cas12f1 gRNA (MF/MS5-1)
cttcactgataaagtggagaaccgcttcaccaaaagctgtttagattagaacttgagtgaaggtgggctgcttgcatcagcctaatgtcgagaagtgctttcttcggaaagtaaccctcgaaacaaattcattt

SEQ ID NO: 115 - RNA, 129 nt, synthetic construct
  source 1..129: mol_type = other RNA; note = Engineered tracrRNA for TnpB or Cas12f1 gRNA (MF/MS5-2)
cttcactgataaagtggagaaccgcttcaccaaaagctttagagaacttgagtgaaggtgggctgcttgcatcagcctaatgtcgagaagtgctttcttcggaaagtaaccctcgaaacaaattcattt

SEQ ID NO: 116 - RNA, 119 nt, synthetic construct
  source 1..119: mol_type = other RNA; note = Engineered tracrRNA for TnpB or Cas12f1 gRNA (MF/MS5-3)
cttcactgataaagtggagaaccgcttcaccaattagttgagtgaaggtgggctgcttgcatcagcctaatgtcgagaagtgctttcttcggaaagtaaccctcgaaacaaattcattt

SEQ ID NO: 117 - RNA, 113 nt, synthetic construct
  source 1..113: mol_type = other RNA; note = Engineered tracrRNA for TnpB or Cas12f1 gRNA (MF/MS5)
cttcactgataaagtggagaaccgcttcacttagagtgaaggtgggctgcttgcatcagcctaatgtcgagaagtgctttcttcggaaagtaaccctcgaaacaaattcattt

SEQ ID NO: 118 - RNA, 118 nt, synthetic construct
  source 1..118: mol_type = other RNA; note = Engineered tracrRNA for TnpB or Cas12f1 gRNA (MF/MS3-3/MS4-1)
accgcttcaccaaaagctgtcccttaggggattagaacttgagtgaaggtgggctgcttgcatcagcctaatgtcgagaagtgctttcttcggaaagtaaccctcgaaacaaattcat

SEQ ID NO: 119 - RNA, 116 nt, synthetic construct
  source 1..116: mol_type = other RNA; note = Engineered tracrRNA for TnpB or Cas12f1 gRNA (MF/MS3-3/MS4-2)
accgcttcaccaaaagctgtcccttaggggattagaacttgagtgaaggtgggctgcttgcatcagcctaatgtcgagaagtgctttcttcggaaagtaaccctcgaaacaaattc

SEQ ID NO: 120 - RNA, 113 nt, synthetic construct
  source 1..113: mol_type = other RNA; note = Engineered tracrRNA for TnpB or Cas12f1 gRNA (MF/MS3-3/MS4-3)
accgcttcaccaaaagctgtcccttaggggattagaacttgagtgaaggtgggctgcttgcatcagcctaatgtcgagaagtgctttcttcggaaagtaaccctcgaaacaaa

SEQ ID NO: 121 - RNA, 127 nt, synthetic construct
  source 1..127: mol_type = other RNA; note = Engineered tracrRNA for TnpB or Cas12f1 gRNA (MF/MS4-3/MS5-1)
cttcactgataaagtggagaaccgcttcaccaaaagctgtttagattagaacttgagtgaaggtgggctgcttgcatcagcctaatgtcgagaagtgctttcttcggaaagtaaccctcgaaacaaa

SEQ ID NO: 122 - RNA, 122 nt, synthetic construct
  source 1..122: mol_type = other RNA; note = Engineered tracrRNA for TnpB or Cas12f1 gRNA (MF/MS4-3/MS5-2)
cttcactgataaagtggagaaccgcttcaccaaaagctttagagaacttgagtgaaggtgggctgcttgcatcagcctaatgtcgagaagtgctttcttcggaaagtaaccctcgaaacaaa

SEQ ID NO: 123 - RNA, 112 nt, synthetic construct
  source 1..112: mol_type = other RNA; note = Engineered tracrRNA for TnpB or Cas12f1 gRNA (MF/MS4-3/MS5-3)
cttcactgataaagtggagaaccgcttcaccaattagttgagtgaaggtgggctgcttgcatcagcctaatgtcgagaagtgctttcttcggaaagtaaccctcgaaacaaa

SEQ ID NO: 124 - RNA, 106 nt, synthetic construct
  source 1..106: mol_type = other RNA; note = Engineered tracrRNA for TnpB or Cas12f1 gRNA (MF/MS4-3/MS5)
cttcactgataaagtggagaaccgcttcacttagagtgaaggtgggctgcttgcatcagcctaatgtcgagaagtgctttcttcggaaagtaaccctcgaaacaaa

SEQ ID NO: 125 - RNA, 114 nt, synthetic construct
  source 1..114: mol_type = other RNA; note = Engineered tracrRNA for TnpB or Cas12f1 gRNA (MF/MS3-3/MS5-1)
accgcttcaccaaaagctgtttagattagaacttgagtgaaggtgggctgcttgcatcagcctaatgtcgagaagtgctttcttcggaaagtaaccctcgaaacaaattcattt

SEQ ID NO: 126 - RNA, 109 nt, synthetic construct
  source 1..109: mol_type = other RNA; note = Engineered tracrRNA for TnpB or Cas12f1 gRNA (MF/MS3-3/MS5-2)
accgcttcaccaaaagctttagagaacttgagtgaaggtgggctgcttgcatcagcctaatgtcgagaagtgctttcttcggaaagtaaccctcgaaacaaattcattt

SEQ ID NO: 127 - RNA, 99 nt, synthetic construct
  source 1..99: mol_type = other RNA; note = Engineered tracrRNA for TnpB or Cas12f1 gRNA (MF/MS3-3/MS5-3)
accgcttcaccaattagttgagtgaaggtgggctgcttgcatcagcctaatgtcgagaagtgctttcttcggaaagtaaccctcgaaacaaattcattt

SEQ ID NO: 128 - RNA, 93 nt, synthetic construct
  source 1..93: mol_type = other RNA; note = Engineered tracrRNA for TnpB or Cas12f1 gRNA (MF/MS3-3/MS5)
accgcttcacttagagtgaaggtgggctgcttgcatcagcctaatgtcgagaagtgctttcttcggaaagtaaccctcgaaacaaattcattt

SEQ ID NO: 129 - RNA, 92 nt, synthetic construct
  source 1..92: mol_type = other RNA; note = Engineered tracrRNA for TnpB or Cas12f1 gRNA (MF/MS3-3/MS4-3/MS5-3)
accgcttcaccaattagttgagtgaaggtgggctgcttgcatcagcctaatgtcgagaagtgctttcttcggaaagtaaccctcgaaacaaa

SEQ ID NO: 130 - RNA, 91 nt, synthetic construct
  source 1..91: mol_type = other RNA; note = Engineered tracrRNA for TnpB or Cas12f1 gRNA (MF/MS3-3/MS4-1/MS5)
accgcttcacttagagtgaaggtgggctgcttgcatcagcctaatgtcgagaagtgctttcttcggaaagtaaccctcgaaacaaattcat

SEQ ID NO: 131 - RNA, 89 nt, synthetic construct
  source 1..89: mol_type = other RNA; note = Engineered tracrRNA for TnpB or Cas12f1 gRNA (MF/MS3-3/MS4-2/MS5)
accgcttcacttagagtgaaggtgggctgcttgcatcagcctaatgtcgagaagtgctttcttcggaaagtaaccctcgaaacaaattc

SEQ ID NO: 132 - RNA, 86 nt, synthetic construct
  source 1..86: mol_type = other RNA; note = Engineered tracrRNA for TnpB or Cas12f1 gRNA (MF/MS3-3/MS4-3/MS5)
accgcttcacttagagtgaaggtgggctgcttgcatcagcctaatgtcgagaagtgctttcttcggaaagtaaccctcgaaacaaa

SEQ ID NO: 133 - RNA, 37 nt, synthetic construct
  source 1..37: mol_type = other RNA; note = Engineered crRNA for TnpB or Cas12f1 gRNA (MS1)
gttgcagaacccgaatagagcaatgaaggaatgcaac

SEQ ID NO: 134 - RNA, 31 nt, synthetic construct
  source 1..31: mol_type = other RNA; note = Engineered crRNA for TnpB or Cas12f1 gRNA (MS1/MS4*-1)
gaacccgaatagagcaatgaaggaatgcaac

SEQ ID NO: 135 - RNA, 25 nt, synthetic construct
  source 1..25: mol_type = other RNA; note = Engineered crRNA for TnpB or Cas12f1 gRNA (MS1/MS4*-2)
gaatagagcaatgaaggaatgcaac

SEQ ID NO: 136 - RNA, 19 nt, synthetic construct
  source 1..19: mol_type = other RNA; note = Engineered crRNA for TnpB or Cas12f1 gRNA (MS1/MS4*-3)
agcaatgaaggaatgcaac

SEQ ID NO: 137 - RNA, 17 nt, synthetic construct
  source 1..17: mol_type = other RNA; note = Engineered crRNA for TnpB or Cas12f1 gRNA (MF)
gaatgaaggaatgcaac

SEQ ID NO: 138 - RNA, 15 nt, synthetic construct
  source 1..15: mol_type = other RNA; note = Engineered crRNA for TnpB or Cas12f1 gRNA (MF/MS4-1)
atgaaggaatgcaac

SEQ ID NO: 139 - RNA, 13 nt, synthetic construct
  source 1..13: mol_type = other RNA; note = Engineered crRNA for TnpB or Cas12f1 gRNA (MF/MS4-2)
gaaggaatgcaac

SEQ ID NO: 140 - RNA, 10 nt, synthetic construct
  source 1..10: mol_type = other RNA; note = Engineered crRNA for TnpB or Cas12f1 gRNA (MF/MS4-3)
ggaatgcaac

SEQ ID NO: 141 - RNA, 68 nt, synthetic construct
  source 1..68: mol_type = other RNA; note = Engineered crRNA for TnpB or Cas12f1 gRNA (MS1/MS2)
  misc_feature 38..57: note = n is a, c, g or u
gttgcagaacccgaatagagcaatgaaggaatgcaacnnnnnnnnnnnnnnnnnnnnttttatttttt

SEQ ID NO: 142 - RNA, 62 nt, synthetic construct
  source 1..62: mol_type = other RNA; note = Engineered crRNA for TnpB or Cas12f1 gRNA (MS1/MS2/MS4*-1)
  misc_feature 32..51: note = n is a, c, g or u
gaacccgaatagagcaatgaaggaatgcaacnnnnnnnnnnnnnnnnnnnnttttatttttt

SEQ ID NO: 143 - RNA, 56 nt, synthetic construct
  source 1..56: mol_type = other RNA; note = Engineered crRNA for TnpB or Cas12f1 gRNA (MS1/MS2/MS4*-2)
  misc_feature 26..45: note = n is a, c, g or u
gaatagagcaatgaaggaatgcaacnnnnnnnnnnnnnnnnnnnnttttatttttt

SEQ ID NO: 144 - RNA, 50 nt, synthetic construct
  source 1..50: mol_type = other RNA; note = Engineered crRNA for TnpB or Cas12f1 gRNA (MS1/MS2/MS4*-3)
  misc_feature 20..39: note = n is a, c, g or u
agcaatgaaggaatgcaacnnnnnnnnnnnnnnnnnnnnttttatttttt

SEQ ID NO: 145 - RNA, 48 nt, synthetic construct
  source 1..48: mol_type = other RNA; note = Engineered crRNA for TnpB or Cas12f1 gRNA (MF/MS2)
  misc_feature 18..37: note = n is a, c, g or u
gaatgaaggaatgcaacnnnnnnnnnnnnnnnnnnnnttttatttttt

SEQ ID NO: 146 - RNA, 46 nt, synthetic construct
  source 1..46: mol_type = other RNA; note = Engineered crRNA for TnpB or Cas12f1 gRNA (MF/MS2/MS4-1)
  misc_feature 16..35: note = n is a, c, g or u
atgaaggaatgcaacnnnnnnnnnnnnnnnnnnnnttttatttttt

SEQ ID NO: 147 - RNA, 44 nt, synthetic construct
  source 1..44: mol_type = other RNA; note = Engineered crRNA for TnpB or Cas12f1 gRNA (MF/MS2/MS4-2)
  misc_feature 14..33: note = n is a, c, g or u
gaaggaatgcaacnnnnnnnnnnnnnnnnnnnnttttatttttt

SEQ ID NO: 148 - RNA, 41 nt, synthetic construct
  source 1..41: mol_type = other RNA; note = Engineered crRNA for TnpB or Cas12f1 gRNA (MF/MS2/MS4-3)
  misc_feature 11..30: note = n is a, c, g or u
ggaatgcaacnnnnnnnnnnnnnnnnnnnnttttatttttt

SEQ ID NO: 149 - RNA, 222 nt, synthetic construct
  source 1..222: mol_type = other RNA; note = Engineered sgRNA with modification of MS1 for TnpB or Cas12f1
  misc_feature 203..222: note = n is a, c, g or u
cttcactgataaagtggagaaccgcttcaccaaaagctgtcccttaggggattagaacttgagtgaaggtgggctgcttgcatcagcctaatgtcgagaagtgctttcttcggaaagtaaccctcgaaacaaattcagtgctcctctccaattctgcacaagaaagttgcagaacccgaatagagcaatgaaggaatgcaacnnnnnnnnnnnnnnnnnnnn

SEQ ID NO: 150 - RNA, 233 nt, synthetic construct
  source 1..233: mol_type = other RNA; note = Engineered sgRNA with modification of MS1/MS2 for TnpB or Cas12f1
  misc_feature 203..222: note = n is a, c, g or u
cttcactgataaagtggagaaccgcttcaccaaaagctgtcccttaggggattagaacttgagtgaaggtgggctgcttgcatcagcctaatgtcgagaagtgctttcttcggaaagtaaccctcgaaacaaattcagtgctcctctccaattctgcacaagaaagttgcagaacccgaatagagcaatgaaggaatgcaacnnnnnnnnnnnnnnnnnnnnttttatttttt

SEQ ID NO: 151 - RNA, 213 nt, synthetic construct
  source 1..213: mol_type = other RNA; note = Engineered sgRNA with modification of MS1/MS2/MS3 for TnpB or Cas12f1
  misc_structure 183..202: note = n is a, c, g or u
accgcttcaccaaaagctgtcccttaggggattagaacttgagtgaaggtgggctgcttgcatcagcctaatgtcgagaagtgctttcttcggaaagtaaccctcgaaacaaattcagtgctcctctccaattctgcacaagaaagttgcagaacccgaatagagcaatgaaggaatgcaacnnnnnnnnnnnnnnnnnnnnttttatttttt

SEQ ID NO: 152 - RNA, 158 nt, synthetic construct
  source 1..158: mol_type = other RNA; note = Engineered sgRNA with modification of MS2/MS3/MS4 for TnpB or Cas12f1
  misc_feature 128..147: note = n is a, c, g or u
accgcttcaccaaaagctgtcccttaggggattagaacttgagtgaaggtgggctgcttgcatcagcctaatgtcgagaagtgctttcttcggaaagtaaccctcgaaacaaagaaaggaatgcaacnnnnnnnnnnnnnnnnnnnnttttatttttt

SEQ ID NO: 153 - RNA, 129 nt, synthetic construct
  source 1..129: mol_type = other RNA; note = Engineered sgRNA with modification of MS2/MS3/MS4/MS5 for TnpB or Cas12f1
  misc_feature 99..118: note = n is a, c, g or u
accgcttcaccgagtgaaggtgggctgcttgcatcagcctaatgtcgagaagtgctttcttcggaaagtaaccctcgaaacaaagaaaggaatgcaacnnnnnnnnnnnnnnnnnnnnttttatttttt

SEQ ID NO: 154 - RNA, 215 nt, synthetic construct
  source 1..215: mol_type = other RNA; note = Engineered sgRNA with modification of MS1/MS3-1 for TnpB or Cas12f1
  misc_feature 196..215: note = n is a, c, g or u
gataaagtggagaaccgcttcaccaaaagctgtcccttaggggattagaacttgagtgaaggtgggctgcttgcatcagcctaatgtcgagaagtgctttcttcggaaagtaaccctcgaaacaaattcagtgctcctctccaattctgcacaagaaagttgcagaacccgaatagagcaatgaaggaatgcaacnnnnnnnnnnnnnnnnnnnn

SEQ ID NO: 155 - RNA, 208 nt, synthetic construct
  source 1..208: mol_type = other RNA; note = Engineered sgRNA with modification of MS1/MS3-2 for TnpB or Cas12f1
  misc_feature 189..208: note = n is a, c, g or u
tggagaaccgcttcaccaaaagctgtcccttaggggattagaacttgagtgaaggtgggctgcttgcatcagcctaatgtcgagaagtgctttcttcggaaagtaaccctcgaaacaaattcagtgctcctctccaattctgcacaagaaagttgcagaacccgaatagagcaatgaaggaatgcaacnnnnnnnnnnnnnnnnnnnn

SEQ ID NO: 156 - RNA, 202 nt, synthetic construct
  source 1..202: mol_type = other RNA; note = Engineered sgRNA with modification of MS1/MS3-3 for TnpB or Cas12f1
  misc_feature 183..202: note = n is a, c, g or u
accgcttcaccaaaagctgtcccttaggggattagaacttgagtgaaggtgggctgcttgcatcagcctaatgtcgagaagtgctttcttcggaaagtaaccctcgaaacaaattcagtgctcctctccaattctgcacaagaaagttgcagaacccgaatagagcaatgaaggaatgcaacnnnnnnnnnnnnnnnnnnnn

SEQ ID NO: 157 - RNA, 209 nt, synthetic construct
  source 1..209: mol_type = other RNA; note = Engineered sgRNA with modification of MS1/MS4*-1 for TnpB or Cas12f1
  misc_feature 190..209: note = n is a, c, g or u
cttcactgataaagtggagaaccgcttcaccaaaagctgtcccttaggggattagaacttgagtgaaggtgggctgcttgcatcagcctaatgtcgagaagtgctttcttcggaaagtaaccctcgaaacaaattcagtgctcctctccaattcgaaagaacccgaatagagcaatgaaggaatgcaacnnnnnnnnnnnnnnnnnnnn

SEQ ID NO: 158 - RNA, 197 nt, synthetic construct
  source 1..197: mol_type = other RNA; note = Engineered sgRNA with modification of MS1/MS4*-2 for TnpB or Cas12f1
  misc_feature 178..197: note = n is a, c, g or u
cttcactgataaagtggagaaccgcttcaccaaaagctgtcccttaggggattagaacttgagtgaaggtgggctgcttgcatcagcctaatgtcgagaagtgctttcttcggaaagtaaccctcgaaacaaattcagtgctcctctcgaaagaatagagcaatgaaggaatgcaacnnnnnnnnnnnnnnnnnnnn

SEQ ID NO: 159 - RNA, 185 nt, synthetic construct
  source 1..185: mol_type = other RNA; note = Engineered sgRNA with modification of MS1/MS4*-3 for TnpB or Cas12f1
  misc_feature 166..185: note = n is a, c, g or u
cttcactgataaagtggagaaccgcttcaccaaaagctgtcccttaggggattagaacttgagtgaaggtgggctgcttgcatcagcctaatgtcgagaagtgctttcttcggaaagtaaccctcgaaacaaattcagtgctgaaaagcaatgaaggaatgcaacnnnnnnnnnnnnnnnnnnnn

SEQ ID NO: 160 - RNA, 216 nt, synthetic construct
  source 1..216: mol_type = other RNA; note = Engineered sgRNA with modification of MS1/MS5-1 for TnpB or Cas12f1
  misc_feature 197..216: note = n is a, c, g or u
cttcactgataaagtggagaaccgcttcaccaaaagctgtttagattagaacttgagtgaaggtgggctgcttgcatcagcctaatgtcgagaagtgctttcttcggaaagtaaccctcgaaacaaattcagtgctcctctccaattctgcacaagaaagttgcagaacccgaatagagcaatgaaggaatgcaacnnnnnnnnnnnnnnnnnnnn

SEQ ID NO: 161 - RNA, 209 nt, synthetic construct
  source 1..209: mol_type = other RNA; note = Engineered sgRNA with modification of MS1/MS5-2 for TnpB or Cas12f1
  misc_feature 190..209: note = n is a, c, g or u
cttcactgataaagtggagaaccgcttcaccaaaagcttaggaacttgagtgaaggtgggctgcttgcatcagcctaatgtcgagaagtgctttcttcggaaagtaaccctcgaaacaaattcagtgctcctctccaattctgcacaagaaagttgcagaacccgaatagagcaatgaaggaatgcaacnnnnnnnnnnnnnnnnnnnn

SEQ ID NO: 162 - RNA, 201 nt, synthetic construct
  source 1..201: mol_type = other RNA; note = Engineered sgRNA with modification of MS1/MS5-3 for TnpB or Cas12f1
  misc_feature 182..201: note = n is a, c, g or u
cttcactgataaagtggagaaccgcttcaccaattagttgagtgaaggtgggctgcttgcatcagcctaatgtcgagaagtgctttcttcggaaagtaaccctcgaaacaaattcagtgctcctctccaattctgcacaagaaagttgcagaacccgaatagagcaatgaaggaatgcaacnnnnnnnnnnnnnnnnnnnn

SEQ ID NO: 163 - RNA, 206 nt, synthetic construct
  source 1..206: mol_type = other RNA; note = Engineered sgRNA with modification of MS1/MS2/MS4*-2 for TnpB or Cas12f1
  misc_feature 178..197: note = n is a, c, g or u
cttcactgataaagtggagaaccgcttcaccaaaagctgtcccttaggggattagaacttgagtgaaggtgggctgcttgcatcagcctaatgtcgagaagtgctttcttcggaaagtaaccctcgaaacaaattcagtgctcctctcgaaagaatagagcaatgaaggaatgcaacnnnnnnnnnnnnnnnnnnnnttttatttt

SEQ ID NO: 164 - RNA, 177 nt, synthetic construct
  source 1..177: mol_type = other RNA; note = Engineered sgRNA with modification of MS1/MS3-3/MS4*-2 for TnpB or Cas12f1
  misc_feature 158..177: note = n is a, c, g or u
accgcttcaccaaaagctgtcccttaggggattagaacttgagtgaaggtgggctgcttgcatcagcctaatgtcgagaagtgctttcttcggaaagtaaccctcgaaacaaattcagtgctcctctcgaaagaatagagcaatgaaggaatgcaacnnnnnnnnnnnnnnnnnnnn

SEQ ID NO: 165 - RNA, 210 nt, synthetic construct
  source 1..210: mol_type = other RNA; note = Engineered sgRNA with modification of MS1/MS2/MS5-3 for TnpB or Cas12f1
  misc_feature 182..201: note = n is a, c, g or u
cttcactgataaagtggagaaccgcttcaccaattagttgagtgaaggtgggctgcttgcatcagcctaatgtcgagaagtgctttcttcggaaagtaaccctcgaaacaaattcagtgctcctctccaattctgcacaagaaagttgcagaacccgaatagagcaatgaaggaatgcaacnnnnnnnnnnnnnnnnnnnnttttatttt

SEQ ID NO: 166 - RNA, 181 nt, synthetic construct
  source 1..181: mol_type = other RNA; note = Engineered sgRNA with modification of MS1/MS3-3/MS5-3 for TnpB or Cas12f1
  misc_feature 162..181: note = n is a, c, g or u
accgcttcaccaattagttgagtgaaggtgggctgcttgcatcagcctaatgtcgagaagtgctttcttcggaaagtaaccctcgaaacaaattcagtgctcctctccaattctgcacaagaaagttgcagaacccgaatagagcaatgaaggaatgcaacnnnnnnnnnnnnnnnnnnnn

SEQ ID NO: 167 - RNA, 176 nt, synthetic construct
  source 1..176: mol_type = other RNA; note = Engineered sgRNA with modification of MS1/MS4*-2/MS5-3 for TnpB or Cas12f1
  misc_feature 157..176: note = n is a, c, g or u
cttcactgataaagtggagaaccgcttcaccaattagttgagtgaaggtgggctgcttgcatcagcctaatgtcgagaagtgctttcttcggaaagtaaccctcgaaacaaattcagtgctcctctcgaaagaatagagcaatgaaggaatgcaacnnnnnnnnnnnnnnnnnnnn

SEQ ID NO: 168 - RNA, 186 nt, synthetic construct
  source 1..186: mol_type = other RNA; note = Engineered sgRNA with modification of MS1/MS2/MS3-3/MS4*-2 for TnpB or Cas12f1
  misc_feature 158..177: note = n is a, c, g or u
accgcttcaccaaaagctgtcccttaggggattagaacttgagtgaaggtgggctgcttgcatcagcctaatgtcgagaagtgctttcttcggaaagtaaccctcgaaacaaattcagtgctcctctcgaaagaatagagcaatgaaggaatgcaacnnnnnnnnnnnnnnnnnnnnttttatttt

SEQ ID NO: 169 - RNA, 190 nt, synthetic construct
  source 1..190: mol_type = other RNA; note = Engineered sgRNA with modification of MS1/MS2/MS3-3/MS5-3 for TnpB or Cas12f1
  misc_feature 162..181: note = n is a, c, g or u
accgcttcaccaattagttgagtgaaggtgggctgcttgcatcagcctaatgtcgagaagtgctttcttcggaaagtaaccctcgaaacaaattcagtgctcctctccaattctgcacaagaaagttgcagaacccgaatagagcaatgaaggaatgcaacnnnnnnnnnnnnnnnnnnnnttttatttt

SEQ ID NO: 170 - RNA, 185 nt, synthetic construct
  source 1..185: mol_type = other RNA; note = Engineered sgRNA with modification of MS1/MS2/MS4*-2/MS5-3 for TnpB or Cas12f1
  misc_feature 157..176: note = n is a, c, g or u
cttcactgataaagtggagaaccgcttcaccaattagttgagtgaaggtgggctgcttgcatcagcctaatgtcgagaagtgctttcttcggaaagtaaccctcgaaacaaattcagtgctcctctcgaaagaatagagcaatgaaggaatgcaacnnnnnnnnnnnnnnnnnnnnttttatttt

SEQ ID NO: 171 - RNA, 156 nt, synthetic construct
  source 1..156: mol_type = other RNA; note = Engineered sgRNA with modification of MS1/MS3-3/MS4*-2/MS5-3 for TnpB or Cas12f1
  misc_feature 137..156: note = n is a, c, g or u
accgcttcaccaattagttgagtgaaggtgggctgcttgcatcagcctaatgtcgagaagtgctttcttcggaaagtaaccctcgaaacaaattcagtgctcctctcgaaagaatagagcaatgaaggaatgcaacnnnnnnnnnnnnnnnnnnnn

SEQ ID NO: 172 - RNA, 165 nt, synthetic construct
  source 1..165: mol_type = other RNA; note = Engineered sgRNA with modification of MS1/MS2/MS3-3/MS4*-2/MS5-3 for TnpB or Cas12f1
  misc_feature 137..156: note = n is a, c, g or u
accgcttcaccaattagttgagtgaaggtgggctgcttgcatcagcctaatgtcgagaagtgctttcttcggaaagtaaccctcgaaacaaattcagtgctcctctcgaaagaatagagcaatgaaggaatgcaacnnnnnnnnnnnnnnnnnnnnttttatttt

SEQ ID NO: 173 - RNA, 181 nt, synthetic construct
  source 1..181: mol_type = other RNA; note = Mature form sgRNA for TnpB or Cas12f1
  misc_feature 162..181: note = n is a, c, g or u
cttcactgataaagtggagaaccgcttcaccaaaagctgtcccttaggggattagaacttgagtgaaggtgggctgcttgcatcagcctaatgtcgagaagtgctttcttcggaaagtaaccctcgaaacaaattcatttgaaagaatgaaggaatgcaacnnnnnnnnnnnnnnnnnnnn

SEQ ID NO: 174 - RNA, 174 nt, synthetic construct
  source 1..174: mol_type = other RNA; note = Mature form sgRNA with modification of MS3-1 for TnpB or Cas12f1
  misc_feature 155..174: note = n is a, c, g or u
gataaagtggagaaccgcttcaccaaaagctgtcccttaggggattagaacttgagtgaaggtgggctgcttgcatcagcctaatgtcgagaagtgctttcttcggaaagtaaccctcgaaacaaattcatttgaaagaatgaaggaatgcaacnnnnnnnnnnnnnnnnnnnn

SEQ ID NO: 175 - RNA, 167 nt, synthetic construct
  source 1..167: mol_type = other RNA; note = Mature form sgRNA with modification of MS3-2 for TnpB or Cas12f1
  misc_feature 148..167: note = n is a, c, g or u
tggagaaccgcttcaccaaaagctgtcccttaggggattagaacttgagtgaaggtgggctgcttgcatcagcctaatgtcgagaagtgctttcttcggaaagtaaccctcgaaacaaattcatttgaaagaatgaaggaatgcaacnnnnnnnnnnnnnnnnnnnn

SEQ ID NO: 176 - RNA, 161 nt, synthetic construct
  source 1..161: mol_type = other RNA; note = Mature form sgRNA with modification of MS3-3 for TnpB or Cas12f1
  misc_feature 142..161: note = n is a, c, g or u
accgcttcaccaaaagctgtcccttaggggattagaacttgagtgaaggtgggctgcttgcatcagcctaatgtcgagaagtgctttcttcggaaagtaaccctcgaaacaaattcatttgaaagaatgaaggaatgcaacnnnnnnnnnnnnnnnnnnnn

SEQ ID NO: 177 - RNA, 177 nt, synthetic construct
  source 1..177: mol_type = other RNA; note = Mature form sgRNA with modification of MS4-1 for TnpB or Cas12f1
  misc_feature 158..177: note = n is a, c, g or u
cttcactgataaagtggagaaccgcttcaccaaaagctgtcccttaggggattagaacttgagtgaaggtgggctgcttgcatcagcctaatgtcgagaagtgctttcttcggaaagtaaccctcgaaacaaattcatgaaaatgaaggaatgcaacnnnnnnnnnnnnnnnnnnnn

SEQ ID NO: 178 - RNA, 173 nt, synthetic construct
  source 1..173: mol_type = other RNA; note = Mature form sgRNA with modification of MS4-2 for TnpB or Cas12f1
  misc_feature 154..173: note = n is a, c, g or u
cttcactgataaagtggagaaccgcttcaccaaaagctgtcccttaggggattagaacttgagtgaaggtgggctgcttgcatcagcctaatgtcgagaagtgctttcttcggaaagtaaccctcgaaacaaattcgaaagaaggaatgcaacnnnnnnnnnnnnnnnnnnnn

SEQ ID NO: 179 - RNA, 167 nt, synthetic construct
  source 1..167: mol_type = other RNA; note = Mature form sgRNA with modification of MS4-3 for TnpB or Cas12f1
  misc_feature 148..167: note = n is a, c, g or u
cttcactgataaagtggagaaccgcttcaccaaaagctgtcccttaggggattagaacttgagtgaaggtgggctgcttgcatcagcctaatgtcgagaagtgctttcttcggaaagtaaccctcgaaacaaagaaaggaatgcaacnnnnnnnnnnnnnnnnnnnn

SEQ ID NO: 180 - RNA, 175 nt, synthetic construct
  source 1..175: mol_type = other RNA; note = Mature form sgRNA with modification of MS5-1 for TnpB or Cas12f1
  misc_feature 156..175: note = n is a, c, g or u
cttcactgataaagtggagaaccgcttcaccaaaagctgtttagattagaacttgagtgaaggtgggctgcttgcatcagcctaatgtcgagaagtgctttcttcggaaagtaaccctcgaaacaaattcatttgaaagaatgaaggaatgcaacnnnnnnnnnnnnnnnnnnnn

SEQ ID NO: 181 - RNA, 170 nt, synthetic construct
  source 1..170: mol_type = other RNA; note = Mature form sgRNA with modification of MS5-2 for TnpB or Cas12f1
  misc_feature 151..170: note = n is a, c, g or u
cttcactgataaagtggagaaccgcttcaccaaaagctttagagaacttgagtgaaggtgggctgcttgcatcagcctaatgtcgagaagtgctttcttcggaaagtaaccctcgaaacaaattcatttgaaagaatgaaggaatgcaacnnnnnnnnnnnnnnnnnnnn

SEQ ID NO: 182 - RNA, 160 nt, synthetic construct
  source 1..160: mol_type = other RNA; note = Mature form sgRNA with modification of MS5-3 for TnpB or Cas12f1
  misc_feature 141..160: note = n is a, c, g or u
cttcactgataaagtggagaaccgcttcaccaattagttgagtgaaggtgggctgcttgcatcagcctaatgtcgagaagtgctttcttcggaaagtaaccctcgaaacaaattcatttgaaagaatgaaggaatgcaacnnnnnnnnnnnnnnnnnnnn

SEQ ID NO: 183 - RNA, 147 nt, synthetic construct
  source 1..147: mol_type = other RNA; note = Mature form sgRNA with modification of MS3-3/MS4-3 for TnpB or Cas12f1
  misc_feature 128..147: note = n is a, c, g or u
accgcttcaccaaaagctgtcccttaggggattagaacttgagtgaaggtgggctgcttgcatcagcctaatgtcgagaagtgctttcttcggaaagtaaccctcgaaacaaagaaaggaatgcaacnnnnnnnnnnnnnnnnnnnn

SEQ ID NO: 184 - RNA, 140 nt, synthetic construct
  source 1..140: mol_type = other RNA; note = Mature form sgRNA with modification of MS3-3/MS5-3 for TnpB or Cas12f1
  misc_feature 121..140: note = n is a, c, g or u
accgcttcaccaattagttgagtgaaggtgggctgcttgcatcagcctaatgtcgagaagtgctttcttcggaaagtaaccctcgaaacaaattcatttgaaagaatgaaggaatgcaacnnnnnnnnnnnnnnnnnnnn

SEQ ID NO: 185 - RNA, 146 nt, synthetic construct
  source 1..146: mol_type = other RNA; note = Mature form sgRNA with modification of MS4-3/MS5-3 for TnpB or Cas12f1
  misc_feature 127..146: note = n is a, c, g or u
cttcactgataaagtggagaaccgcttcaccaattagttgagtgaaggtgggctgcttgcatcagcctaatgtcgagaagtgctttcttcggaaagtaaccctcgaaacaaagaaaggaatgcaacnnnnnnnnnnnnnnnnnnnn

SEQ ID NO: 186 - RNA, 126 nt, synthetic construct
  source 1..126: mol_type = other RNA; note = Mature form sgRNA with modification of MS3-3/MS4-3/MS5-3 for TnpB or Cas12f1
  misc_feature 107..126: note = n is a, c, g or u
accgcttcaccaattagttgagtgaaggtgggctgcttgcatcagcctaatgtcgagaagtgctttcttcggaaagtaaccctcgaaacaaagaaaggaatgcaacnnnnnnnnnnnnnnnnnnnn

SEQ ID NO: 187 - RNA, 10 nt, synthetic construct
  source 1..10: mol_type = other RNA; note = The additional sequence for TnpB or Cas12f1 gRNA
ataaaggtga

SEQ ID NO: 188 - RNA, 37 nt, synthetic construct
  source 1..37: mol_type = other RNA; note = The additional sequence for TnpB or Cas12f1 gRNA
ctgatgagtccgtgaggacgaaacgagtaagctcgtc

SEQ ID NO: 189 - RNA, 37 nt, synthetic construct
  source 1..37: mol_type = other RNA; note = The additional sequence for TnpB or Cas12f1 gRNA
ctgctcgaatgagcaaagcaggagtgcctgagtagtc

SEQ ID NO: 190 - DNA, 20 bp, synthetic construct
  source 1..20: mol_type = other DNA; note = F102 -protospacer
aggttgtctcctcattagag

SEQ ID NO: 191 - DNA, 20 bp, synthetic construct
  source 1..20: mol_type = other DNA; note = F104 -protospacer
atattcttagaatcgttcac

SEQ ID NO: 192 - DNA, 20 bp, synthetic construct
  source 1..20: mol_type = other DNA; note = F108 -protospacer
ccaccaatcttctggttata

SEQ ID NO: 193 - DNA, 20 bp, synthetic construct
  source 1..20: mol_type = other DNA; note = F109 -protospacer
tagacaacagactcaagagc

SEQ ID NO: 194 - DNA, 20 bp, synthetic construct
  source 1..20: mol_type = other DNA; note = F110 -protospacer
actgactactccccaagtat

SEQ ID NO: 195 - DNA, 20 bp, synthetic construct
  source 1..20: mol_type = other DNA; note = F111 -protospacer
gggccttatctccagtttct

SEQ ID NO: 196 - DNA, 20 bp, synthetic construct
  source 1..20: mol_type = other DNA; note = F114 -protospacer
taaacgcctggctagtaaga

SEQ ID NO: 197 - DNA, 20 bp, synthetic construct
  source 1..20: mol_type = other DNA; note = F115 -protospacer
taaaaacagtaatacctaac

SEQ ID NO: 198 - DNA, 20 bp, synthetic construct
  source 1..20: mol_type = other DNA; note = F118 -protospacer
ccttgcttactgcttattgc

SEQ ID NO: 199 - DNA, 20 bp, synthetic construct
  source 1..20: mol_type = other DNA; note = F119 -protospacer
ttcagtactagcaataagca

SEQ ID NO: 200 - DNA, 20 bp, synthetic construct
  source 1..20: mol_type = other DNA; note = F121 -protospacer
tttaatgactttgaaacagt

SEQ ID NO: 201 - DNA, 20 bp, synthetic construct
  source 1..20: mol_type = other DNA; note = F123 -protospacer
aaacagtatttcatgtctaa

SEQ ID NO: 202 - DNA, 20 bp, synthetic construct
  source 1..20: mol_type = other DNA; note = F124 -protospacer
gacatgaaatactgtttcaa

SEQ ID NO: 203 - DNA, 20 bp, synthetic construct
  source 1..20: mol_type = other DNA; note = F128 -protospacer
agaaaatattgtatcttggt

SEQ ID NO: 204 - DNA, 20 bp, synthetic construct
  source 1..20: mol_type = other DNA; note = F130 -protospacer
tttcagattgttagtaaact

SEQ ID NO: 205 - DNA, 20 bp, synthetic construct
  source 1..20: mol_type = other DNA; note = F131 -protospacer
tactgggagcagtttatcat

SEQ ID NO: 206 - DNA, 20 bp, synthetic construct
  source 1..20: mol_type = other DNA; note = F133 -protospacer
atttccctagggtccagctt

SEQ ID NO: 207 - DNA, 20 bp, synthetic construct
  source 1..20: mol_type = other DNA; note = F134 -protospacer
aagctggaccctagggaaat

SEQ ID NO: 208 - DNA, 20 bp, synthetic construct
  source 1..20: mol_type = other DNA; note = F135 -protospacer
aaattcccttgaataggaag

SEQ ID NO: 209 - DNA, 20 bp, synthetic construct
  source 1..20: mol_type = other DNA; note = F136 -protospacer
aatcagaaagaagatcttat

SEQ ID NO: 210 - DNA, 20 bp, synthetic construct
  source 1..20: mol_type = other DNA; note = F138 -protospacer
ttcaagaaaaaacaaaggca

SEQ ID NO: 211 - DNA, 20 bp, synthetic construct
  source 1..20: mol_type = other DNA; note = F140 -protospacer
ccacttccacaatgtatatg

SEQ ID NO: 212 - DNA, 20 bp, synthetic construct
  source 1..20: mol_type = other DNA; note = F141 -protospacer
acttaagttacttgtccagg

SEQ ID NO: 213 - DNA, 20 bp, synthetic construct
  source 1..20: mol_type = other DNA; note = F142 -protospacer
ctcattctcatgcctggaca

SEQ ID NO: 214 - DNA, 20 bp, synthetic construct
  source 1..20: mol_type = other DNA; note = F143 -protospacer
aaaaattgttaaatgtatat

SEQ ID NO: 215 - DNA, 20 bp, synthetic construct
  source 1..20: mol_type = other DNA; note = F147 -protospacer
attgaagagtaacaatttga

SEQ ID NO: 216 - DNA, 20 bp, synthetic construct
  source 1..20: mol_type = other DNA; note = F148 -protospacer
acttattgttattgaaattg

SEQ ID NO: 217 - DNA, 20 bp, synthetic construct
  source 1..20: mol_type = other DNA; note = F43 -protospacer
gtatcaattcacaccagcaa

SEQ ID NO: 218 - DNA, 20 bp, synthetic construct
  source 1..20: mol_type = other DNA; note = R52 -protospacer
ctctcctagaccatttccca

SEQ ID NO: 219 - DNA, 20 bp, synthetic construct
  source 1..20: mol_type = other DNA; note = R55 -protospacer
ctgagagagaaacagttgcc

SEQ ID NO: 220 - DNA, 20 bp, synthetic construct
  source 1..20: mol_type = other DNA; note = R56 -protospacer
tatccttgattatacttagg

SEQ ID NO: 221 - DNA, 20 bp, synthetic construct
  source 1..20: mol_type = other DNA; note = R57 -protospacer
cattaatttatatccttgat

SEQ ID NO: 222 - DNA, 20 bp, synthetic construct
  source 1..20: mol_type = other DNA; note = R58 -protospacer
ttatttgcattaatttatat

SEQ ID NO: 223 - DNA, 20 bp, synthetic construct
  source 1..20: mol_type = other DNA; note = R59 -protospacer
actgagacaactattcttgt

SEQ ID NO: 224 - DNA, 20 bp, synthetic construct
  source 1..20: mol_type = other DNA; note = R60 -protospacer
gtaaatttaactgagacaac

SEQ ID NO: 225 - DNA, 20 bp, synthetic construct
  source 1..20: mol_type = other DNA; note = R61 -protospacer
aaataccaggttgtttagta

SEQ ID NO: 226 - DNA, 20 bp, synthetic construct
  source 1..20: mol_type = other DNA; note = R62 -protospacer
taccaaataagtcactcaac

SEQ ID NO: 227 - DNA, 20 bp, synthetic construct
  source 1..20: mol_type = other DNA; note = R63 -protospacer
aatgtaaatagctcagttga

SEQ ID NO: 228 - DNA, 20 bp, synthetic construct
  source 1..20: mol_type = other DNA; note = R64 -protospacer
gcactacgcagcccaacata

SEQ ID NO: 229 - DNA, 20 bp, synthetic construct
  source 1..20: mol_type = other DNA; note = R65 -protospacer
attctgcaatatgttgggct

SEQ ID NO: 230 - DNA, 20 bp, synthetic construct
  source 1..20: mol_type = other DNA; note = R66 -protospacer
ccttctccaatgataaggat

SEQ ID NO: 231 - DNA, 20 bp, synthetic construct
  source 1..20: mol_type = other DNA; note = R68 -protospacer
agttatagctctctttcaat

SEQ ID NO: 232 - DNA, 20 bp, synthetic construct
  source 1..20: mol_type = other DNA; note = R69 -protospacer
aaattaccctagatcttaaa

SEQ ID NO: 233 - DNA, 20 bp, synthetic construct
  source 1..20: mol_type = other DNA; note = R70 -protospacer
tgcaatgccatgttcaaatg

SEQ ID NO: 234 - DNA, 20 bp, synthetic construct
  source 1..20: mol_type = other DNA; note = R71 -protospacer
aacatggcattgcataaatg

SEQ ID NO: 235 - DNA, 20 bp, synthetic construct
  source 1..20: mol_type = other DNA; note = R73 -protospacer
ccaaatggattacactgagg

SEQ ID NO: 236 - DNA, 20 bp, synthetic construct
  source 1..20: mol_type = other DNA; note = R74 -protospacer
gtaaaattatgacatcaact

SEQ ID NO: 237 - DNA, 20 bp, synthetic construct
  source 1..20: mol_type = other DNA; note = R75 -protospacer
cctagctagatcaaatatac

SEQ ID NO: 238 - DNA, 20 bp, synthetic construct
  source 1..20: mol_type = other DNA; note = R76 -protospacer
atctagctaggtaaaccata

SEQ ID NO: 239 - DNA, 20 bp, synthetic construct
  source 1..20: mol_type = other DNA; note = R77 -protospacer
tatttgtgaatgattaagaa

SEQ ID NO: 240 - DNA, 20 bp, synthetic construct
  source 1..20: mol_type = other DNA; note = R79 -protospacer
atgtataacaattccaacat

SEQ ID NO: 241 - DNA, 20 bp, synthetic construct
  source 1..20: mol_type = other DNA; note = R82 -protospacer
gaaaggcttgaaagctgtta

SEQ ID NO: 242 - DNA, 20 bp, synthetic construct
  source 1..20: mol_type = other DNA; note = R84 -protospacer
tatttctttagaaaggcttg

SEQ ID NO: 243 - DNA, 20 bp, synthetic construct
  source 1..20: mol_type = other DNA; note = R85 -protospacer
atacctaaataccttcagca

SEQ ID NO: 244 - DNA, 20 bp, synthetic construct
  source 1..20: mol_type = other DNA; note = R86 -protospacer
aaaaaacaagaagtgaggca

SEQ ID NO: 245 - DNA, 20 bp, synthetic construct
  source 1..20: mol_type = other DNA; note = R89 -protospacer
taaaataaacttcaccaatt

SEQ ID NO: 246 - DNA, 20 bp, synthetic construct
  source 1..20: mol_type = other DNA; note = R90 -protospacer
caaagaaattccccttactc

SEQ ID NO: 247 - DNA, 20 bp, synthetic construct
  source 1..20: mol_type = other DNA; note = R91 -protospacer
ttcctatggaattggtgaag

SEQ ID NO: 248 - DNA, 20 bp, synthetic construct
  source 1..20: mol_type = other DNA; note = R92 -protospacer
aaggccttgagcttgaatac

SEQ ID NO: 249 - DNA, 20 bp, synthetic construct
  source 1..20: mol_type = other DNA; note = R93 -protospacer
aatgcaggttgtttactatc

SEQ ID NO: 250 - DNA, 20 bp, synthetic construct
  source 1..20: mol_type = other DNA; note = R94 -protospacer
caaatgatgattgtggtcaa

SEQ ID NO: 251 - DNA, 20 bp, synthetic construct
  source 1..20: mol_type = other DNA; note = R95 -protospacer
caaatggcactgaattcagg

SEQ ID NO: 252 - DNA, 20 bp, synthetic construct
  source 1..20: mol_type = other DNA; note = R97 -protospacer
tatacatccatatccataac

SEQ ID NO: 253 - DNA, 20 bp, synthetic construct
  source 1..20: mol_type = other DNA; note = R98 -protospacer
catatatttatatacatcca

SEQ ID NO: 254 - DNA, 20 bp, synthetic construct
  source 1..20: mol_type = other DNA; note = R99 -protospacer
cttctgctttaaaaaaagta

SEQ ID NO: 255 - DNA, 20 bp, synthetic construct
  source 1..20: mol_type = other DNA; note = F1 -protospacer
tcatcccaatggcatattta

SEQ ID NO: 256 - DNA, 20 bp, synthetic construct
  source 1..20: mol_type = other DNA; note = F2 -protospacer
gtcatcatgaaccattctct

SEQ ID NO: 257 - DNA, 20 bp, synthetic construct
  source 1..20: mol_type = other DNA; note = F3 -protospacer
agtctcaggccctggccttg

SEQ ID NO: 258 - DNA, 20 bp, synthetic construct
  source 1..20: mol_type = other DNA; note = F4 -protospacer
gaaaaagacagaaaggaaga

SEQ ID NO: 259 - DNA, 20 bp, synthetic construct
  source 1..20: mol_type = other DNA; note = F5 -protospacer
ttgaaatttagtgtgacatg

SEQ ID NO: 260 - DNA, 20 bp, synthetic construct
  source 1..20: mol_type = other DNA; note = F6 -protospacer
gtgtgacatgatcatttcca

SEQ ID NO: 261 - DNA, 20 bp, synthetic construct
  source 1..20: mol_type = other DNA; note = F7 -protospacer
accctcaaataagagcagag

SEQ ID NO: 262 - DNA, 20 bp, synthetic construct
  source 1..20: mol_type = other DNA; note = F8 -protospacer
agggtcaaattttcaataag

SEQ ID NO: 263 - DNA, 20 bp, synthetic construct
  source 1..20: mol_type = other DNA; note = F9 -protospacer
aaaagtgacttattgaaaat

SEQ ID NO: 264 - DNA, 20 bp, synthetic construct
  source 1..20: mol_type = other DNA; note = F10 -protospacer
aaaaagcattttctgacact

SEQ ID NO: 265 - DNA, 20 bp, synthetic construct
  source 1..20: mol_type = other DNA; note = F11 -protospacer
ggaggatttcaagcttatgg

SEQ ID NO: 266 - DNA, 20 bp, synthetic construct
  source 1..20: mol_type = other DNA; note = F12 -protospacer
ggaacactccatccacattt

SEQ ID NO: 267 - DNA, 20 bp, synthetic construct
  source 1..20: mol_type = other DNA; note = F13 -protospacer
ccagtcagcctggtgttctg

SEQ ID NO: 268 - DNA, 20 bp, synthetic construct
  source 1..20: mol_type = other DNA; note = F14 -protospacer
atttagctctcttttcatcc

SEQ ID NO: 269 - DNA, 20 bp, synthetic construct
  source 1..20: mol_type = other DNA; note = F15 -protospacer
gctctcttttcatcctcaca

SEQ ID NO: 270 - DNA, 20 bp, synthetic construct
  source 1..20: mol_type = other DNA; note = F16 -protospacer
gctcctttcctggaatccct

SEQ ID NO: 271 - DNA, 20 bp, synthetic construct
  source 1..20: mol_type = other DNA; note = F17 -protospacer
cttccatgatttcttctcct

SEQ ID NO: 272 - DNA, 20 bp, synthetic construct
  source 1..20: mol_type = other DNA; note = F18 -protospacer
tgtcacagtccaggagaaga

SEQ ID NO: 273 - DNA, 20 bp, synthetic construct
  source 1..20: mol_type = other DNA; note = F19 -protospacer
cattacatttaattctttct

SEQ ID NO: 274 - DNA, 20 bp, synthetic construct
  source 1..20: mol_type = other DNA; note = F20 -protospacer
attctttctagaaagagcct

SEQ ID NO: 275 - DNA, 20 bp, synthetic construct
  source 1..20: mol_type = other DNA; note = F21 -protospacer
tttctcaaagctatctgact

SEQ ID NO: 276 - DNA, 20 bp, synthetic construct
  source 1..20: mol_type = other DNA; note = F22 -protospacer
ttgcctcactgttactgcct

SEQ ID NO: 277 - DNA, 20 bp, synthetic construct
  source 1..20: mol_type = other DNA; note = F23 -protospacer
tgtcacgaaacaatgattga

SEQ ID NO: 278 - DNA, 20 bp, synthetic construct
  source 1..20: mol_type = other DNA; note = F24 -protospacer
attgtcagagagaataaaaa

SEQ ID NO: 279 - DNA, 20 bp, synthetic construct
  source 1..20: mol_type = other DNA; note = F25 -protospacer
ttctctctgacaattaaaac

SEQ ID NO: 280 - DNA, 20 bp, synthetic construct
  source 1..20: mol_type = other DNA; note = F26 -protospacer
atcaatgcagacagaaaaaa

SEQ ID NO: 281 - DNA, 20 bp, synthetic construct
  source 1..20: mol_type = other DNA; note = R1 -protospacer
acatctatgagcctcagtta

SEQ ID NO: 282 - DNA, 20 bp, synthetic construct
  source 1..20: mol_type = other DNA; note = R2 -protospacer
aatccttgttctgctactta

SEQ ID NO: 283 - DNA, 20 bp, synthetic construct
  source 1..20: mol_type = other DNA; note = R3 -protospacer
attcctaagcttgtgttatt

SEQ ID NO: 284 - DNA, 20 bp, synthetic construct
  source 1..20: mol_type = other DNA; note = R4 -protospacer
gtgatttgtatgtagatgta

SEQ ID NO: 285 - DNA, 20 bp, synthetic construct
  source 1..20: mol_type = other DNA; note = R5 -protospacer
tatgtagatgtagatgtagt

SEQ ID NO: 286 - DNA, 20 bp, synthetic construct
  source 1..20: mol_type = other DNA; note = R6 -protospacer
tggttgctatgtactgatac

SEQ ID NO: 287 - DNA, 20 bp, synthetic construct
  source 1..20: mol_type = other DNA; note = R7 -protospacer
caataccatattgagttata

SEQ ID NO: 288 - DNA, 20 bp, synthetic construct
  source 1..20: mol_type = other DNA; note = R8 -protospacer
gtaaataaaagtcctgggag

SEQ ID NO: 289 - DNA, 20 bp, synthetic construct
  source 1..20: mol_type = other DNA; note = R9 -protospacer
tttaccaaaggaaacaatat

SEQ ID NO: 290 - DNA, 20 bp, synthetic construct
  source 1..20: mol_type = other DNA; note = R10 -protospacer
ccaaaggaaacaatatttta

SEQ ID NO: 291 - DNA, 20 bp, synthetic construct
  source 1..20: mol_type = other DNA; note = R11 -protospacer
aacattataaaatattgttt

SEQ ID NO: 292 - DNA, 20 bp, synthetic construct
  source 1..20: mol_type = other DNA; note = R12 -protospacer
taatgtttaaagcccaggtt

SEQ ID NO: 293 - DNA, 20 bp, synthetic construct
  source 1..20: mol_type = other DNA; note = R13 -protospacer
aagcccaggttttgaagtta

SEQ ID NO: 294 - DNA, 20 bp, synthetic construct
  source 1..20: mol_type = other DNA; note = R14 -protospacer
aacccagacaatgtaacttc

SEQ ID NO: 295 - DNA, 20 bp, synthetic construct
  source 1..20: mol_type = other DNA; note = R15 -protospacer
aagttacattgtctgggttc

SEQ ID NO: 296 - DNA, 20 bp, synthetic construct
  source 1..20: mol_type = other DNA; note = R16 -protospacer
tagctagataaacttgggct

SEQ ID NO: 297 - DNA, 20 bp, synthetic construct
  source 1..20: mol_type = other DNA; note = R17 -protospacer
tctagctataaaatggggat

SEQ ID NO: 298 - DNA, 20 bp, synthetic construct
  source 1..20: mol_type = other DNA; note = R18 -protospacer
tcatcaggattaagttggtt

SEQ ID NO: 299 - DNA, 20 bp, synthetic construct
  source 1..20: mol_type = other DNA; note = R19 -protospacer
ttcaatactagcagtaagca

SEQ ID NO: 300 - DNA, 20 bp, synthetic construct
  source 1..20: mol_type = other DNA; note = R20 -protospacer
ccttgcttactgcttactgc

SEQ ID NO: 301 - DNA, 20 bp, synthetic construct
  source 1..20: mol_type = other DNA; note = R21 -protospacer
gttccaccacgaactctaga

SEQ ID NO: 302 - DNA, 20 bp, synthetic construct
  source 1..20: mol_type = other DNA; note = R22 -protospacer
cataatacaaatgccatcat

SEQ ID NO: 303 - DNA, 20 bp, synthetic construct
  source 1..20: mol_type = other DNA; note = R23 -protospacer
tattatgcaaactgtatatc

SEQ ID NO: 304 - DNA, 20 bp, synthetic construct
  source 1..20: mol_type = other DNA; note = R24 -protospacer
tgagtccagcatttagggaa

SEQ ID NO: 305 - DNA, 20 bp, synthetic construct
  source 1..20: mol_type = other DNA; note = R25 -protospacer
gggaagccattgatgtgctc

SEQ ID NO: 306 - DNA, 20 bp, synthetic construct
  source 1..20: mol_type = other DNA; note = R26 -protospacer
gagaactctggagactactg

SEQ ID NO: 307 - DNA, 20 bp, synthetic construct
  source 1..20: mol_type = other DNA; note = R27 -protospacer
tttagagaactctggagact

SEQ ID NO: 308 - DNA, 20 bp, synthetic construct
  source 1..20: mol_type = other DNA; note = R28 -protospacer
atgccccctcacagagatcg

SEQ ID NO: 309 - DNA, 20 bp, synthetic construct
  source 1..20: mol_type = other DNA; note = R29 -protospacer
aagacgatctctgtgagggg

SEQ ID NO: 310 - DNA, 20 bp, synthetic construct
  source 1..20: mol_type = other DNA; note = R30 -protospacer
acctatatttaaagacgatc

SEQ ID NO: 311 - DNA, 20 bp, synthetic construct
  source 1..20: mol_type = other DNA; note = R31 -protospacer
aatataggtcaaaaactaat

SEQ ID NO: 312 - RNA, 19 nt, synthetic construct
  source 1..19: mol_type = other RNA; note = Spacer 1 for dystrophin(w/o U-tail)
ctcattctcatgcctggac

SEQ ID NO: 313 - RNA, 20 nt, synthetic construct
  source 1..20: mol_type = other RNA; note = Spacer 2 for dystrophin(w/o U-tail)
ctcattctcatgcctggaca

SEQ ID NO: 314 - RNA, 21 nt, synthetic construct
  source 1..21: mol_type = other RNA; note = Spacer 3 for dystrophin(w/o U-tail)
ctcattctcatgcctggacaa

SEQ ID NO: 315 - RNA, 22 nt, synthetic construct
  source 1..22: mol_type = other RNA; note = Spacer 4 for dystrophin(w/o U-tail)
ctcattctcatgcctggacaag

SEQ ID NO: 316 - RNA, 24 nt, synthetic construct
  source 1..24: mol_type = other RNA; note = Spacer 5 for dystrophin(w/o U-tail)
ctcattctcatgcctggacaagta

SEQ ID NO: 317 - RNA, 25 nt, synthetic construct
  source 1..25: mol_type = other RNA; note = Spacer 6 for dystrophin(w/o U-tail)
ctcattctcatgcctggacaagtaa

SEQ ID NO: 318 - RNA, 19 nt, synthetic construct
  source 1..19: mol_type = other RNA; note = Spacer 7 for dystrophin(w/o U-tail)
ctcattctcatgcctggac

SEQ ID NO: 319 - RNA, 20 nt, synthetic construct
  source 1..20: mol_type = other RNA; note = Spacer 8 for dystrophin(w/o U-tail)
ctcattctcatgcctggaca

SEQ ID NO: 320 - RNA, 21 nt, synthetic construct
  source 1..21: mol_type = other RNA; note = Spacer 9 for dystrophin(w/o U-tail)
ctcattctcatgcctggacaa

SEQ ID NO: 321 - RNA, 22 nt, synthetic construct
  source 1..22: mol_type = other RNA; note = Spacer 10 for dystrophin(w/o U-tail)
ctcattctcatgcctggacaag

SEQ ID NO: 322 - RNA, 24 nt, synthetic construct
  source 1..24: mol_type = other RNA; note = Spacer 11 for dystrophin(w/o U-tail)
ctcattctcatgcctggacaagta

SEQ ID NO: 323 - RNA, 25 nt, synthetic construct
  source 1..25: mol_type = other RNA; note = Spacer 12 for dystrophin(w/o U-tail)
ctcattctcatgcctggacaagtaa

SEQ ID NO: 324 - RNA, 19 nt, synthetic construct
  source 1..19: mol_type = other RNA; note = Spacer 13 for dystrophin(w/o U-tail)
ctctcctagaccatttccc

SEQ ID NO: 325 - RNA, 20 nt, synthetic construct
  source 1..20: mol_type = other RNA; note = Spacer 14 for dystrophin(w/o U-tail)
ctctcctagaccatttccca

SEQ ID NO: 326 - RNA, 21 nt, synthetic construct
  source 1..21: mol_type = other RNA; note = Spacer 15 for dystrophin(w/o U-tail)
ctctcctagaccatttcccac

SEQ ID NO: 327 - RNA, 22 nt, synthetic construct
  source 1..22: mol_type = other RNA; note = Spacer 16 for dystrophin(w/o U-tail)
ctctcctagaccatttcccacc

SEQ ID NO: 328 - RNA, 23 nt, synthetic construct
  source 1..23: mol_type = other RNA; note = Spacer 17 for dystrophin(w/o U-tail)
ctctcctagaccatttcccacca

SEQ ID NO: 329 - RNA, 24 nt, synthetic construct
  source 1..24: mol_type = other RNA; note = Spacer 18 for dystrophin(w/o U-tail)
ctctcctagaccatttcccaccag

SEQ ID NO: 330 - RNA, 19 nt, synthetic construct
  source 1..19: mol_type = other RNA; note = Spacer 19 for dystrophin(w/o U-tail)
ctctcctagaccatttccc

SEQ ID NO: 331 - RNA, 20 nt, synthetic construct
  source 1..20: mol_type = other RNA; note = Spacer 20 for dystrophin(w/o U-tail)
ctctcctagaccatttccca

SEQ ID NO: 332 - RNA, 21 nt, synthetic construct
  source 1..21: mol_type = other RNA; note = Spacer 21 for dystrophin(w/o U-tail)
ctctcctagaccatttcccac

SEQ ID NO: 333 - RNA, 22 nt, synthetic construct
  source 1..22: mol_type = other RNA; note = Spacer 22 for dystrophin(w/o U-tail)
ctctcctagaccatttcccacc

SEQ ID NO: 334 - RNA, 23 nt, synthetic construct
  source 1..23: mol_type = other RNA; note = Spacer 23 for dystrophin(w/o U-tail)
ctctcctagaccatttcccacca

SEQ ID NO: 335 - RNA, 24 nt, synthetic construct
  source 1..24: mol_type = other RNA; note = Spacer 24 for dystrophin(w/o U-tail)
ctctcctagaccatttcccaccag

SEQ ID NO: 336 - RNA, 28 nt, synthetic construct
  source 1..28: mol_type = other RNA; note = Spacer 1 for dystrophin(w/ U-tail)
ctcattctcatgcctggacttttatttt

SEQ ID NO: 337 - RNA, 29 nt, synthetic construct
  source 1..29: mol_type = other RNA; note = Spacer 2 for dystrophin(w/ U-tail)
ctcattctcatgcctggacattttatttt

SEQ ID NO: 338 - RNA, 30 nt, synthetic construct
  source 1..30: mol_type = other RNA; note = Spacer 3 for dystrophin(w/ U-tail)
ctcattctcatgcctggacaattttatttt

SEQ ID NO: 339 - RNA, 31 nt, synthetic construct
  source 1..31: mol_type = other RNA; note = Spacer 4 for dystrophin(w/ U-tail)
ctcattctcatgcctggacaagttttatttt

SEQ ID NO: 340 - RNA, 33 nt, synthetic construct
  source 1..33: mol_type = other RNA; note = Spacer 5 for dystrophin(w/ U-tail)
ctcattctcatgcctggacaagtattttatttt

SEQ ID NO: 341 - RNA, 34 nt, synthetic construct
  source 1..34: mol_type = other RNA; note = Spacer 6 for dystrophin(w/ U-tail)
ctcattctcatgcctggacaagtaattttatttt

SEQ ID NO: 342 - RNA, 23 nt, synthetic construct
  source 1..23: mol_type = other RNA; note = Spacer 7 for dystrophin(w/ U-tail)
ctcattctcatgcctggactttt

SEQ ID NO: 343 - RNA, 24 nt, synthetic construct
  source 1..24: mol_type = other RNA; note = Spacer 8 for dystrophin(w/ U-tail)
ctcattctcatgcctggacatttt

SEQ ID NO: 344 - RNA, 25 nt, synthetic construct
  source 1..25: mol_type = other RNA; note = Spacer 9 for dystrophin(w/ U-tail)
ctcattctcatgcctggacaatttt

SEQ ID NO: 345 - RNA, 26 nt, synthetic construct
  source 1..26: mol_type = other RNA; note = Spacer 10 for dystrophin(w/ U-tail)
ctcattctcatgcctggacaagtttt

SEQ ID NO: 346 - RNA, 28 nt, synthetic construct
  source 1..28: mol_type = other RNA; note = Spacer 11 for dystrophin(w/ U-tail)
ctcattctcatgcctggacaagtatttt

SEQ ID NO: 347 - RNA, 29 nt, synthetic construct
  source 1..29: mol_type = other RNA; note = Spacer 12 for dystrophin(w/ U-tail)
ctcattctcatgcctggacaagtaatttt

SEQ ID NO: 348 - RNA, 28 nt, synthetic construct
  source 1..28: mol_type = other RNA; note = Spacer 13 for dystrophin(w/ U-tail)
ctctcctagaccatttcccttttatttt

SEQ ID NO: 349 - RNA, 29 nt, synthetic construct
  source 1..29: mol_type = other RNA; note = Spacer 14 for dystrophin(w/ U-tail)
ctctcctagaccatttcccattttatttt

SEQ ID NO: 350 - RNA, 30 nt, synthetic construct
  source 1..30: mol_type = other RNA; note = Spacer 15 for dystrophin(w/ U-tail)
ctctcctagaccatttcccacttttatttt

SEQ ID NO: 351 - RNA, 31 nt, synthetic construct
  source 1..31: mol_type = other RNA; note = Spacer 16 for dystrophin(w/ U-tail)
ctctcctagaccatttcccaccttttatttt

SEQ ID NO: 352 - RNA, 32 nt, synthetic construct
  source 1..32: mol_type = other RNA; note = Spacer 17 for dystrophin(w/ U-tail)
ctctcctagaccatttcccaccattttatttt

SEQ ID NO: 353 - RNA, 33 nt, synthetic construct
  source 1..33: mol_type = other RNA; note = Spacer 18 for dystrophin(w/ U-tail)
ctctcctagaccatttcccaccagttttatttt

SEQ ID NO: 354 - RNA, 23 nt, synthetic construct
  source 1..23: mol_type = other RNA; note = Spacer 19 for dystrophin(w/ U-tail)
ctctcctagaccatttccctttt

SEQ ID NO: 355 - RNA, 24 nt, synthetic construct
  source 1..24: mol_type = other RNA; note = Spacer 20 for dystrophin(w/ U-tail)
ctctcctagaccatttcccatttt

SEQ ID NO: 356 - RNA, 25 nt, synthetic construct
  source 1..25: mol_type = other RNA; note = Spacer 21 for dystrophin(w/ U-tail)
ctctcctagaccatttcccactttt

SEQ ID NO: 357 - RNA, 26 nt, synthetic construct
  source 1..26: mol_type = other RNA; note = Spacer 22 for dystrophin(w/ U-tail)
ctctcctagaccatttcccacctttt

SEQ ID NO: 358 - RNA, 27 nt, synthetic construct
  source 1..27: mol_type = other RNA; note = Spacer 23 for dystrophin(w/ U-tail)
ctctcctagaccatttcccaccatttt

SEQ ID NO: 359 - RNA, 28 nt, synthetic construct
  source 1..28: mol_type = other RNA; note = Spacer 24 for dystrophin(w/ U-tail)
ctctcctagaccatttcccaccagtttt

SEQ ID NO: 360 - RNA, 47 nt, synthetic construct
  source 1..47: mol_type = other RNA; note = shRNA for ATM1-1
ggagccagatagtttgtatttcaagagaatacaaactatctggctcc

SEQ ID NO: 361 - RNA, 47 nt, synthetic construct
  source 1..47: mol_type = other RNA; note = shRNA for ATM1-2
gcaagcagctgaaacaaatttcaagagaatttgtttcagctgcttgc

SEQ ID NO: 362 - RNA, 47 nt, synthetic construct
  source 1..47: mol_type = other RNA; note = shRNA for ATM1-3
ggagctgattgtagcaacattcaagagatgttgctacaatcagctcc

SEQ ID NO: 363 - RNA, 47 nt, synthetic construct
  source 1..47: mol_type = other RNA; note = shRNA for ATM1-4
gcacagaagtgcctccaatttcaagagaattggaggcacttctgtgc

SEQ ID NO: 364 - RNA, 47 nt, synthetic construct
  source 1..47: mol_type = other RNA; note = shRNA for ATM1-5
ggacatagtttctgggagattcaagagatctcccagaaactatgtcc

SEQ ID NO: 365 - RNA, 47 nt, synthetic construct
  source 1..47: mol_type = other RNA; note = shRNA for XRCC4-1
ggatgacactggcacattattcaagagataatgtgccagtgtcatcc

SEQ ID NO: 366 - RNA, 47 nt, synthetic construct
  source 1..47: mol_type = other RNA; note = shRNA for XRCC4-2
ggagagtactgatgaggaattcaagagattcctcatcagtactctcc

SEQ ID NO: 367 - RNA, 47 nt, synthetic construct
  source 1..47: mol_type = other RNA; note = shRNA for XRCC4-3
gaatccaccttgtttctgattcaagagatcagaaacaaggtggattc

SEQ ID NO: 368 - RNA, 47 nt, synthetic construct
  source 1..47: mol_type = other RNA; note = shRNA for XRCC4-4
gtacaagtatcttgggagattcaagagatctcccaagatacttgtac

SEQ ID NO: 369 - RNA, 47 nt, synthetic construct
  source 1..47: mol_type = other RNA; note = shRNA for XRCC4-5
gaatgcagctcaagaacgattcaagagatcgttcttgagctgcattc

SEQ ID NO: 370 - RNA, 47 nt, synthetic construct
  source 1..47: mol_type = other RNA; note = shRNA for XLF-1
gcatgagtctggcattacattcaagagatgtaatgccagactcatgc

SEQ ID NO: 371 - RNA, 47 nt, synthetic construct
  source 1..47: mol_type = other RNA; note = shRNA for XLF-2
gaaagccctttgtcatgaattcaagagattcatgacaaagggctttc

SEQ ID NO: 372 - RNA, 47 nt, synthetic construct
  source 1..47: mol_type = other RNA; note = shRNA for XLF-3
gaacagtgcttccctgcaattcaagagattgcagggaagcactgttc

SEQ ID NO: 373 - RNA, 47 nt, synthetic construct
  source 1..47: mol_type = other RNA; note = shRNA for XLF-4
ggaaagacctagagatccattcaagagatggatctctaggtctttcc

SEQ ID NO: 374 - RNA, 47 nt, synthetic construct
  source 1..47: mol_type = other RNA; note = shRNA for XLF-5
gtatggcagtcaccacacattcaagagatgtgtggtgactgccatac

SEQ ID NO: 375 - RNA, 47 nt, synthetic construct
  source 1..47: mol_type = other RNA; note = shRNA for XRCC6-1
gcagcattgtgcagatacattcaagagatgtatctgcacaatgctgc

SEQ ID NO: 376 - RNA, 47 nt, synthetic construct
  source 1..47: mol_type = other RNA; note = shRNA for XRCC6-2
gcaggaacatccctccttattcaagagataaggagggatgttcctgc

SEQ ID NO: 377 - RNA, 47 nt, synthetic construct
  source 1..47: mol_type = other RNA; note = shRNA for XRCC6-3
gcagtgctctgctcatcaattcaagagattgatgagcagagcactgc

SEQ ID NO: 378 - RNA, 47 nt, synthetic construct
  source 1..47: mol_type = other RNA; note = shRNA for XRCC6-4
ggatcatgctgttcaccaattcaagagattggtgaacagcatgatcc

SEQ ID NO: 379 - RNA, 47 nt, synthetic construct
  source 1..47: mol_type = other RNA; note = shRNA for XRCC6-5
ggatctgactactcactcattcaagagatgagtgagtagtcagatcc

SEQ ID NO: 380 - RNA, 47 nt, synthetic construct
  source 1..47: mol_type = other RNA; note = shRNA for LIG4-1
gcacaaagatggagatgtattcaagagatacatctccatctttgtgc

SEQ ID NO: 381 - RNA, 47 nt, synthetic construct
  source 1..47: mol_type = other RNA; note = shRNA for LIG4-2
gcagacacgtactgtgtaattcaagagattacacagtacgtgtctgc

SEQ ID NO: 382 - RNA, 47 nt, synthetic construct
  source 1..47: mol_type = other RNA; note = shRNA for LIG4-3
ggagcagactcctgaagaattcaagagattcttcaggagtctgctcc

SEQ ID NO: 383 - RNA, 47 nt, synthetic construct
  source 1..47: mol_type = other RNA; note = shRNA for LIG4-4
ggaggattctgatctgcaattcaagagattgcagatcagaatcctcc

SEQ ID NO: 384 - RNA, 47 nt, synthetic construct
  source 1..47: mol_type = other RNA; note = shRNA for LIG4-5
gcatgatccttctgtaggattcaagagatcctacagaaggatcatgc

SEQ ID NO: 385 - RNA, 47 nt, synthetic construct
  source 1..47: mol_type = other RNA; note = shRNA for DCLRE1C-1
ggagactcctacccagatattcaagagatatctgggtaggagtctcc

SEQ ID NO: 386 - RNA, 47 nt, synthetic construct
  source 1..47: mol_type = other RNA; note = shRNA for DCLRE1C-2
ggacaaagctgactacagattcaagagatctgtagtcagctttgtcc

SEQ ID NO: 387 - RNA, 47 nt, synthetic construct
  source 1..47: mol_type = other RNA; note = shRNA for DCLRE1C-3
gcagagctctcgtttcacattcaagagatgtgaaacgagagctctgc

SEQ ID NO: 388 - RNA, 47 nt, synthetic construct
  source 1..47: mol_type = other RNA; note = shRNA for DCLRE1C-4
ggactctgatggagaatcattcaagagatgattctccatcagagtcc

SEQ ID NO: 389 - RNA, 47 nt, synthetic construct
  source 1..47: mol_type = other RNA; note = shRNA for DCLRE1C-5
gcagaattcttcccagtcattcaagagatgactgggaagaattctgc

SEQ ID NO: 390 - protein, 249 aa, synthetic construct
  source 1..249: note = N-term 249aa extension
MVSKGEELFTGVVPILVELDGDVNGHKFSVSGEGEGDATYGKLTLKFICTTGKLPVPWPTLVTTLTYGVQCFSRYPDHMKQHDFFKSAMPEGYVQERTIFFKDDGNYKTRAEVKFEGDTLVNRIELKGIDFKEDGNILGHKLEYNYNSHNVYIMADKQKNGIKVNFKIRHNIEDGSVQLADHYQQNTPIGDGPVLLPDNHYLSTQSALSKDPNEKRDHMVLLEFVTAAGITLGMDELYKSGLRSRAQAL

SEQ ID NO: 391 - protein, 248 aa, synthetic construct
  source 1..248: note = C-term 248aa extension
RARDPPVATMVSKGEELFTGVVPILVELDGDVNGHKFSVSGEGEGDATYGKLTLKFICTTGKLPVPWPTLVTTLTYGVQCFSRYPDHMKQHDFFKSAMPEGYVQERTIFFKDDGNYKTRAEVKFEGDTLVNRIELKGIDFKEDGNILGHKLEYNYNSHNVYIMADKQKNGIKVNFKIRHNIEDGSVQLADHYQQNTPIGDGPVLLPDNHYLSTQSALSKDPNEKRDHMVLLEFVTAAGITLGMDELYK

SEQ ID NO: 392 - protein, 557 aa, synthetic construct
  source 1..557: note = Engineered CWCas12f1 (S170T)
MGEKSSRRRRNGKSGAWTAAITSCVGGKMAKNTITKTLKLRIVRPYNSAEVEKIVADEKNNREKIALEKNKDKVKEACSKHLKVAAYCTTQVERNACLFCKARKLDDKFYQKLRGQFPDAVFWQEISEIFRQLQKQAAEIYNQSLIELYYEIFIKGKGIANASSVEHYLTDVCYTRAAELFKNAAIASGLRSKIKSNFRLKELKNMKSGLPTTKSDNFPIPLVKQKGGQYTGFEISNHNSDFIIKIPFGRWQVKKEIDKYRPWEKFDFEQVQKSPKPISLLLSTQRRKRNKGWSKDEGTEAEIKKVMNGDYQTSYIEVKRGSKIGEKSAWMLNLSIDVPKIDKGVDPSIIGGIDVGVKSPLVCAINNAFSRYSISDNDLFHFNKKMFARRRILLKKNRHKRAGHGAKNKLKPITILTEKSERFRKKLIERWACEIADFFIKNKVGTVQMENLESMKRKEDSYFNIRLRGFWPYAEMQNKIEFKLKQYGIEIRKVAPNNTSKTCSKCGHLNNYFNFEYRKKNKFPHFKCEKCNFKENADYNAALNISNPKLKSTKEEP

SEQ ID NO: 393 - protein, 557 aa, synthetic construct
  source 1..557: note = Engineered CWCas12f1 (S188Q)
MGEKSSRRRRNGKSGAWTAAITSCVGGKMAKNTITKTLKLRIVRPYNSAEVEKIVADEKNNREKIALEKNKDKVKEACSKHLKVAAYCTTQVERNACLFCKARKLDDKFYQKLRGQFPDAVFWQEISEIFRQLQKQAAEIYNQSLIELYYEIFIKGKGIANASSVEHYLSDVCYTRAAELFKNAAIAQGLRSKIKSNFRLKELKNMKSGLPTTKSDNFPIPLVKQKGGQYTGFEISNHNSDFIIKIPFGRWQVKKEIDKYRPWEKFDFEQVQKSPKPISLLLSTQRRKRNKGWSKDEGTEAEIKKVMNGDYQTSYIEVKRGSKIGEKSAWMLNLSIDVPKIDKGVDPSIIGGIDVGVKSPLVCAINNAFSRYSISDNDLFHFNKKMFARRRILLKKNRHKRAGHGAKNKLKPITILTEKSERFRKKLIERWACEIADFFIKNKVGTVQMENLESMKRKEDSYFNIRLRGFWPYAEMQNKIEFKLKQYGIEIRKVAPNNTSKTCSKCGHLNNYFNFEYRKKNKFPHFKCEKCNFKENADYNAALNISNPKLKSTKEEP

SEQ ID NO: 394 - protein, 557 aa, synthetic construct
  source 1..557: note = Engineered CWCas12f1 (S188H)
MGEKSSRRRRNGKSGAWTAAITSCVGGKMAKNTITKTLKLRIVRPYNSAEVEKIVADEKNNREKIALEKNKDKVKEACSKHLKVAAYCTTQVERNACLFCKARKLDDKFYQKLRGQFPDAVFWQEISEIFRQLQKQAAEIYNQSLIELYYEIFIKGKGIANASSVEHYLSDVCYTRAAELFKNAAIAHGLRSKIKSNFRLKELKNMKSGLPTTKSDNFPIPLVKQKGGQYTGFEISNHNSDFIIKIPFGRWQVKKEIDKYRPWEKFDFEQVQKSPKPISLLLSTQRRKRNKGWSKDEGTEAEIKKVMNGDYQTSYIEVKRGSKIGEKSAWMLNLSIDVPKIDKGVDPSIIGGIDVGVKSPLVCAINNAFSRYSISDNDLFHFNKKMFARRRILLKKNRHKRAGHGAKNKLKPITILTEKSERFRKKLIERWACEIADFFIKNKVGTVQMENLESMKRKEDSYFNIRLRGFWPYAEMQNKIEFKLKQYGIEIRKVAPNNTSKTCSKCGHLNNYFNFEYRKKNKFPHFKCEKCNFKENADYNAALNISNPKLKSTKEEP

SEQ ID NO: 395 - protein, 557 aa, synthetic construct
  source 1..557: note = Engineered CWCas12f1 (S188K)
MGEKSSRRRRNGKSGAWTAAITSCVGGKMAKNTITKTLKLRIVRPYNSAEVEKIVADEKNNREKIALEKNKDKVKEACSKHLKVAAYCTTQVERNACLFCKARKLDDKFYQKLRGQFPDAVFWQEISEIFRQLQKQAAEIYNQSLIELYYEIFIKGKGIANASSVEHYLSDVCYTRAAELFKNAAIAKGLRSKIKSNFRLKELKNMKSGLPTTKSDNFPIPLVKQKGGQYTGFEISNHNSDFIIKIPFGRWQVKKEIDKYRPWEKFDFEQVQKSPKPISLLLSTQRRKRNKGWSKDEGTEAEIKKVMNGDYQTSYIEVKRGSKIGEKSAWMLNLSIDVPKIDKGVDPSIIGGIDVGVKSPLVCAINNAFSRYSISDNDLFHFNKKMFARRRILLKKNRHKRAGHGAKNKLKPITILTEKSERFRKKLIERWACEIADFFIKNKVGTVQMENLESMKRKEDSYFNIRLRGFWPYAEMQNKIEFKLKQYGIEIRKVAPNNTSKTCSKCGHLNNYFNFEYRKKNKFPHFKCEKCNFKENADYNAALNISNPKLKSTKEEP

SEQ ID NO: 396 - protein, 557 aa, synthetic construct
  source 1..557: note = Engineered CWCas12f1 (R191K)
MGEKSSRRRRNGKSGAWTAAITSCVGGKMAKNTITKTLKLRIVRPYNSAEVEKIVADEKNNREKIALEKNKDKVKEACSKHLKVAAYCTTQVERNACLFCKARKLDDKFYQKLRGQFPDAVFWQEISEIFRQLQKQAAEIYNQSLIELYYEIFIKGKGIANASSVEHYLSDVCYTRAAELFKNAAIASGLKSKIKSNFRLKELKNMKSGLPTTKSDNFPIPLVKQKGGQYTGFEISNHNSDFIIKIPFGRWQVKKEIDKYRPWEKFDFEQVQKSPKPISLLLSTQRRKRNKGWSKDEGTEAEIKKVMNGDYQTSYIEVKRGSKIGEKSAWMLNLSIDVPKIDKGVDPSIIGGIDVGVKSPLVCAINNAFSRYSISDNDLFHFNKKMFARRRILLKKNRHKRAGHGAKNKLKPITILTEKSERFRKKLIERWACEIADFFIKNKVGTVQMENLESMKRKEDSYFNIRLRGFWPYAEMQNKIEFKLKQYGIEIRKVAPNNTSKTCSKCGHLNNYFNFEYRKKNKFPHFKCEKCNFKENADYNAALNISNPKLKSTKEEP

SEQ ID NO: 397 - protein, 557 aa, synthetic construct
  source 1..557: note = Engineered CWCas12f1 (Q225T)
MGEKSSRRRRNGKSGAWTAAITSCVGGKMAKNTITKTLKLRIVRPYNSAEVEKIVADEKNNREKIALEKNKDKVKEACSKHLKVAAYCTTQVERNACLFCKARKLDDKFYQKLRGQFPDAVFWQEISEIFRQLQKQAAEIYNQSLIELYYEIFIKGKGIANASSVEHYLSDVCYTRAAELFKNAAIASGLRSKIKSNFRLKELKNMKSGLPTTKSDNFPIPLVKTKGGQYTGFEISNHNSDFIIKIPFGRWQVKKEIDKYRPWEKFDFEQVQKSPKPISLLLSTQRRKRNKGWSKDEGTEAEIKKVMNGDYQTSYIEVKRGSKIGEKSAWMLNLSIDVPKIDKGVDPSIIGGIDVGVKSPLVCAINNAFSRYSISDNDLFHFNKKMFARRRILLKKNRHKRAGHGAKNKLKPITILTEKSERFRKKLIERWACEIADFFIKNKVGTVQMENLESMKRKEDSYFNIRLRGFWPYAEMQNKIEFKLKQYGIEIRKVAPNNTSKTCSKCGHLNNYFNFEYRKKNKFPHFKCEKCNFKENADYNAALNISNPKLKSTKEEP

SEQ ID NO: 398 - protein, 557 aa, synthetic construct
  source 1..557: note = Engineered CWCas12f1 (Q225F)
MGEKSSRRRRNGKSGAWTAAITSCVGGKMAKNTITKTLKLRIVRPYNSAEVEKIVADEKNNREKIALEKNKDKVKEACSKHLKVAAYCTTQVERNACLFCKARKLDDKFYQKLRGQFPDAVFWQEISEIFRQLQKQAAEIYNQSLIELYYEIFIKGKGIANASSVEHYLSDVCYTRAAELFKNAAIASGLRSKIKSNFRLKELKNMKSGLPTTKSDNFPIPLVKFKGGQYTGFEISNHNSDFIIKIPFGRWQVKKEIDKYRPWEKFDFEQVQKSPKPISLLLSTQRRKRNKGWSKDEGTEAEIKKVMNGDYQTSYIEVKRGSKIGEKSAWMLNLSIDVPKIDKGVDPSIIGGIDVGVKSPLVCAINNAFSRYSISDNDLFHFNKKMFARRRILLKKNRHKRAGHGAKNKLKPITILTEKSERFRKKLIERWACEIADFFIKNKVGTVQMENLESMKRKEDSYFNIRLRGFWPYAEMQNKIEFKLKQYGIEIRKVAPNNTSKTCSKCGHLNNYFNFEYRKKNKFPHFKCEKCNFKENADYNAALNISNPKLKSTKEEP

SEQ ID NO: 399 - protein, 557 aa, synthetic construct
  source 1..557: note = Engineered CWCas12f1 (Q272K)
MGEKSSRRRRNGKSGAWTAAITSCVGGKMAKNTITKTLKLRIVRPYNSAEVEKIVADEKNNREKIALEKNKDKVKEACSKHLKVAAYCTTQVERNACLFCKARKLDDKFYQKLRGQFPDAVFWQEISEIFRQLQKQAAEIYNQSLIELYYEIFIKGKGIANASSVEHYLSDVCYTRAAELFKNAAIASGLRSKIKSNFRLKELKNMKSGLPTTKSDNFPIPLVKQKGGQYTGFEISNHNSDFIIKIPFGRWQVKKEIDKYRPWEKFDFEQVKKSPKPISLLLSTQRRKRNKGWSKDEGTEAEIKKVMNGDYQTSYIEVKRGSKIGEKSAWMLNLSIDVPKIDKGVDPSIIGGIDVGVKSPLVCAINNAFSRYSISDNDLFHFNKKMFARRRILLKKNRHKRAGHGAKNKLKPITILTEKSERFRKKLIERWACEIADFFIKNKVGTVQMENLESMKRKEDSYFNIRLRGFWPYAEMQNKIEFKLKQYGIEIRKVAPNNTSKTCSKCGHLNNYFNFEYRKKNKFPHFKCEKCNFKENADYNAALNISNPKLKSTKEEP

SEQ ID NO: 400 - RNA, 20 nt, synthetic construct
  source 1..20: mol_type = other RNA; note = shRNA for human XRCC4-1
gtgatgacactggcacatta

SEQ ID NO: 401 - RNA, 20 nt, synthetic construct
  source 1..20: mol_type = other RNA; note = shRNA for human XRCC4-2
gtgagagtactgatgaggaa

SEQ ID NO: 402 - RNA, 19 nt, synthetic construct
  source 1..19: mol_type = other RNA; note = shRNA for human XRCC4-3
gaatccaccttgtttctga

SEQ ID NO: 403 - RNA, 20 nt, synthetic construct
  source 1..20: mol_type = other RNA; note = shRNA for human XRCC4-4
gctacaagtatcttgggaga

SEQ ID NO: 404 - RNA, 20 nt, synthetic construct
  source 1..20: mol_type = other RNA; note = shRNA for human XRCC4-5
gaaatgcagctcaagaacga

SEQ ID NO: 405 - RNA, 19 nt, synthetic construct
  source 1..19: mol_type = other RNA; note = shRNA for human XLF-1
gcatgagtctggcattaca

SEQ ID NO: 406 - RNA, 19 nt, synthetic construct
  source 1..19: mol_type = other RNA; note = shRNA for human XLF-2
gaaagccctttgtcatgaa

SEQ ID NO: 407 - RNA, 19 nt, synthetic construct
  source 1..19: mol_type = other RNA; note = shRNA for human XLF-3
aaacagtgcttccctgcaa

SEQ ID NO: 408 - RNA, 20 nt, synthetic construct
  source 1..20: mol_type = other RNA; note = shRNA for human XLF-4
gtgaaagacctagagatcca

SEQ ID NO: 409 - RNA, 20 nt, synthetic construct
  source 1..20: mol_type = other RNA; note = shRNA for human XLF-5
gatatggcagtcaccacaca

SEQ ID NO: 410 - RNA, 19 nt, synthetic construct
  source 1..19: mol_type = other RNA; note = shRNA for human XRCC6-1
gcagcattgtgcagataca

SEQ ID NO: 411 - RNA, 19 nt, synthetic construct
  source 1..19: mol_type = other RNA; note = shRNA for human XRCC6-2
gcaggaacatccctcctta

SEQ ID NO: 412 - RNA, 20 nt, synthetic construct
  source 1..20: mol_type = other RNA; note = shRNA for human XRCC6-3
gtcagtgctctgctcatcaa

SEQ ID NO: 413 - RNA, 19 nt, synthetic construct
  source 1..19: mol_type = other RNA; note = shRNA for human XRCC6-4
ggatcatgctgttcaccaa

SEQ ID NO: 414 - RNA, 19 nt, synthetic construct
  source 1..19: mol_type = other RNA; note = shRNA for human XRCC6-5
ggatctgactactcactca

SEQ ID NO: 415 - RNA, 19 nt, synthetic construct
  source 1..19: mol_type = other RNA; note = shRNA for human LIG4-1
gcacaaagatggagatgta

SEQ ID NO: 416 - RNA, 20 nt, synthetic construct
  source 1..20: mol_type = other RNA; note = shRNA for human LIG4-2
gccagacacgtactgtgtaa

SEQ ID NO: 417 - RNA, 20 nt, synthetic construct
  source 1..20: mol_type = other RNA; note = shRNA for human LIG4-3
gcgagcagactcctgaagaa

SEQ ID NO: 418 - RNA, 19 nt, synthetic construct
  source 1..19: mol_type = other RNA; note = shRNA for human LIG4-4
agaggattctgatctgcaa

SEQ ID NO: 419 - RNA, 19 nt, synthetic construct
  source 1..19: mol_type = other RNA; note = shRNA for human LIG4-5
gcatgatccttctgtagga

SEQ ID NO: 420 - RNA, 20 nt, synthetic construct
  source 1..20: mol_type = other RNA; note = shRNA for human DCLRE1C-1
gcgagactcctacccagata

SEQ ID NO: 421 - RNA, 19 nt, synthetic construct
  source 1..19: mol_type = other RNA; note = shRNA for human DCLRE1C-2
ggacaaagctgactacaga

SEQ ID NO: 422 - RNA, 19 nt, synthetic construct
  source 1..19: mol_type = other RNA; note = shRNA for human DCLRE1C-3
gcagagctctcgtttcaca

SEQ ID NO: 423 - RNA, 20 nt, synthetic construct
  source 1..20: mol_type = other RNA; note = shRNA for human DCLRE1C-4
gtgactctgatggagaatca

SEQ ID NO: 424 - RNA, 20 nt, synthetic construct
  source 1..20: mol_type = other RNA; note = shRNA for human DCLRE1C-5
gccagaattcttcccagtca

SEQ ID NO: 425 - RNA, 19 nt, synthetic construct
  source 1..19: mol_type = other RNA; note = shRNA for human ATM1-1
ggagccagatagtttgtat

SEQ ID NO: 426 - RNA, 19 nt, synthetic construct
  source 1..19: mol_type = other RNA; note = shRNA for human ATM1-2
gcaagcagctgaaacaaat

SEQ ID NO: 427 - RNA, 19 nt, synthetic construct
  source 1..19: mol_type = other RNA; note = shRNA for human ATM1-3
ggagctgattgtagcaaca

SEQ ID NO: 428 - RNA, 19 nt, synthetic construct
  source 1..19: mol_type = other RNA; note = shRNA for human ATM1-4
gcacagaagtgcctccaat

SEQ ID NO: 429 - RNA, 19 nt, synthetic construct
  source 1..19: mol_type = other RNA; note = shRNA for human ATM1-5
ggacatagtttctgggaga

SEQ ID NO: 430 - RNA, 19 nt, synthetic construct
  source 1..19: mol_type = other RNA; note = shRNA for human ATM1-6
gaacttcagtggaccttca

SEQ ID NO: 431 - RNA, 20 nt, synthetic construct
  source 1..20: mol_type = other RNA; note = scrambled-1 shRNA
gttctccgaacgtgtcacgt

SEQ ID NO: 432 - RNA, 22 nt, synthetic construct
  source 1..22: mol_type = other RNA; note = scrambled-2 shRNA
gcaacaagatgaagagcaccaa

SEQ ID NO: 433 - RNA, 19 nt, synthetic construct
  source 1..19: mol_type = other RNA; note = shRNA for mouse DCLRE1C-1
gaagaccagtgctaatcta

SEQ ID NO: 434 - RNA, 19 nt, synthetic construct
  source 1..19: mol_type = other RNA; note = shRNA for mouse DCLRE1C-2
ggaccttgatgtgctaaca

SEQ ID NO: 435 - RNA, 19 nt, synthetic construct
  source 1..19: mol_type = other RNA; note = shRNA for mouse DCLRE1C-3
gcaccgcaagccttctata

SEQ ID NO: 436 - RNA, 19 nt, synthetic construct
  source 1..19: mol_type = other RNA; note = shRNA for mouse DCLRE1C-4
gaaactggcaacaggtcaa

SEQ ID NO: 437 - RNA, 19 nt, synthetic construct
  source 1..19: mol_type = other RNA; note = shRNA for mouse DCLRE1C-5
ggatcatgagggagtaaga

SEQ ID NO: 438 - RNA, 19 nt, synthetic construct
  source 1..19: mol_type = other RNA; note = shRNA for mouse DCLRE1C-6
gaagtgttagactattaca

SEQ ID NO: 439 - RNA, 19 nt, synthetic construct
  source 1..19: mol_type = other RNA; note = shRNA for mouse DCLRE1C-7
ggacagtgcacctgactaa

SEQ ID NO: 440 - RNA, 19 nt, synthetic construct
  source 1..19: mol_type = other RNA; note = shRNA for mouse DCLRE1C-8
gaatgtatgggtactgtca

SEQ ID NO: 441 - RNA, 19 nt, synthetic construct
  source 1..19: mol_type = other RNA; note = shRNA for mouse DCLRE1C-9
gaaggtgtaagggtctgaa

SEQ ID NO: 442 - RNA, 20 nt, synthetic construct
  source 1..20: mol_type = other RNA; note = shRNA for mouse DCLRE1C-10
gaatggagcttctgcactct

SEQ ID NO: 443 - RNA, 20 nt, synthetic construct
  source 1..20: mol_type = other RNA; note = shRNA for mouse DCLRE1C-11
gcttatggctacgagtattt

SEQ ID NO: 444 - RNA, 20 nt, synthetic construct
  source 1..20: mol_type = other RNA; note = shRNA for mouse DCLRE1C-12
gagctgggagttcaggttca

SEQ ID NO: 445 - RNA, 19 nt, synthetic construct
  source 1..19: mol_type = other RNA; note = shRNA for mouse DCLRE1C-13
gcatcaagccatctaccat

SEQ ID NO: 446 - RNA, 22 nt, synthetic construct
  source 1..22: mol_type = other RNA; note = scrambled-3 shRNA
cagagctaactcagatagtact

SEQ ID NO: 447 - DNA, 24 bp, synthetic construct
  source 1..24: mol_type = other DNA; note = primer_E51_LD_F for qPCR
tgtcatgaataagagtttggctca

SEQ ID NO: 448 - DNA, 22 bp, synthetic construct
  source 1..22: mol_type = other DNA; note = primer_E51_LD_R for qPCR
aggttgtgtcaccagagtaaca

SEQ ID NO: 449 - DNA, 22 bp, synthetic construct
  source 1..22: mol_type = other DNA; note = primer_18s_rRNA-F for qPCR
tcaactttcgatggtagtcgcc

SEQ ID NO: 450 - DNA, 24 bp, synthetic construct
  source 1..24: mol_type = other DNA; note = primer_18s_rRNA-R for qPCR
ggcctcgaaagagtcctgtattgt

SEQ ID NO: 451 - DNA, 20 bp, synthetic construct
  source 1..20: mol_type = other DNA; note = primer_hATM-F for qRT-PCR
ggacagtggaggcacaaaat

SEQ ID NO: 452 - DNA, 20 bp, synthetic construct
  source 1..20: mol_type = other DNA; note = primer_hATM-R for qRT-PCR
gtgtcgaagacagctggtga

SEQ ID NO: 453 - DNA, 20 bp, synthetic construct
  source 1..20: mol_type = other DNA; note = primer_hXRCC6-F for qRT-PCR
cgggaaacaaatgaaccagt

SEQ ID NO: 454 - DNA, 20 bp, synthetic construct
  source 1..20: mol_type = other DNA; note = primer_hXRCC6-R for qRT-PCR
tgaaacccatgagcatcaaa

SEQ ID NO: 455 - DNA, 20 bp, synthetic construct
  source 1..20: mol_type = other DNA; note = primer_hLIG4-F for qRT-PCR
caccttgcgttttccacgaa

SEQ ID NO: 456 - DNA, 22 bp, synthetic construct
  source 1..22: mol_type = other DNA; note = primer_hLIG4-R for qRT-PCR
cagatgccttccccctaagttg

SEQ ID NO: 457 - DNA, 20 bp, synthetic construct
  source 1..20: mol_type = other DNA; note = primer_hXRCC4-F for qRT-PCR
ctgatggtcattcagcatgg

SEQ ID NO: 458 - DNA, 20 bp, synthetic construct
  source 1..20: mol_type = other DNA; note = primer_hXRCC4-R for qRT-PCR
tcctgctcctgacaacaatg

SEQ ID NO: 459 - DNA, 20 bp, synthetic construct
  source 1..20: mol_type = other DNA; note = primer_hLIG4-F for qRT-PCR
tctctggcctccccttctat

SEQ ID NO: 460 - DNA, 20 bp, synthetic construct
  source 1..20: mol_type = other DNA; note = primer_hLIG4-R for qRT-PCR
tagctccctcacttggcact

SEQ ID NO: 461 - DNA, 20 bp, synthetic construct
  source 1..20: mol_type = other DNA; note = primer_hDCLRE1C-F for qRT-PCR
aattccaagtcgggaggagt

SEQ ID NO: 462 - DNA, 20 bp, synthetic construct
  source 1..20: mol_type = other DNA; note = primer_hDCLRE1C-R for qRT-PCR
ggatctgagtgttgcggtct

SEQ ID NO: 463 - DNA, 21 bp, synthetic construct
  source 1..21: mol_type = other DNA; note = primer_GAPDH-F for qRT-PCR
ggaaggactcatgaccacagt

SEQ ID NO: 464 - DNA, 19 bp, synthetic construct
  source 1..19: mol_type = other DNA; note = primer_GAPDH-R for qRT-PCR
cagtgagcttcccgttcag

SEQ ID NO: 465 - DNA, 22 bp, synthetic construct
  source 1..22: mol_type = other DNA; note = primer_18s_rRNA-F for qRT-PCR
tcaactttcgatggtagtcgcc

SEQ ID NO: 466 - DNA, 24 bp, synthetic construct
  source 1..24: mol_type = other DNA; note = primer_18s_rRNA-R for qRT-PCR
ggcctcgaaagagtcctgtattgt

SEQ ID NO: 467 - DNA, 19 bp, synthetic construct
  source 1..19: mol_type = other DNA; note = primer_mDclrelc-F for qRT-PCR
gcttcgggtgagaaggaag

SEQ ID NO: 468 - DNA, 20 bp, synthetic construct
  source 1..20: mol_type = other DNA; note = primer_mDclrelc-R for qRT-PCR
tgccagtctgaagtctcctg

SEQ ID NO: 469 - RNA, 21 nt, synthetic construct
  source 1..21: mol_type = other RNA; note = scrambled-1 shRNA for mouse
cctaaggttaagtcgccctcg

SEQ ID NO: 470 - RNA, 22 nt, synthetic construct
  source 1..22: mol_type = other RNA; note = scrambled-3 shRNA
cagagctaactcagatagtact

SEQ ID NO: 471 - DNA, 21 bp, synthetic construct
  source 1..21: mol_type = other DNA; note = F68-protospacer for SaCas9
gtgtattgcttgtactactca

SEQ ID NO: 472 - DNA, 21 bp, synthetic construct
  source 1..21: mol_type = other DNA; note = R84-protospacer for SaCas9
gtgttattacttgctactgca

SEQ ID NO: 473 - RNA, 47 nt, synthetic construct
  source 1..47: mol_type = other RNA; note = shRNA for ATM1-6
gaacttcagtggaccttcattcaagagatgaaggtccactgaagttc